European Patent Application EP 4 233 546 A2, published August 30, 2023. Title: ALTERING MICROBIAL POPULATIONS & MODIFYING MICROBIOTA. Applicant: SNIPR TECHNOLOGIES LIMITED. Application EP 22194479.6, filed May 6, 2016. The sequence listing filed with the application follows.

SEQUENCE LISTING (122 sequences)

SEQ ID NO: 1-19 - skipped (19 entries)

SEQ ID NO: 20 - DNA, 10 bp, unidentified
  source 1..10: mol_type = other DNA; note = Bacterial
acgatttgag

SEQ ID NO: 21 - skipped

SEQ ID NO: 22 - DNA, 10 bp, unidentified
  source 1..10: mol_type = other DNA; note = Bacterial
ttcatttgag

SEQ ID NO: 23 - DNA, 10 bp, unidentified
  source 1..10: mol_type = other DNA; note = Bacterial
atcatttgag

SEQ ID NO: 24 - DNA, 11 bp, unidentified
  source 1..11: mol_type = other DNA; note = Bacterial
tttcatttgag

SEQ ID NO: 25 - DNA, 11 bp, unidentified
  source 1..11: mol_type = other DNA; note = Bacterial
aatcatttgag

SEQ ID NO: 26 - DNA, 12 bp, unidentified
  source 1..12: mol_type = other DNA; note = Bacterial
aattcatttgag

SEQ ID NO: 27 - DNA, 12 bp, unidentified
  source 1..12: mol_type = other DNA; note = Bacterial
aaatcatttgag

SEQ ID NO: 28 - DNA, 13 bp, unidentified
  source 1..13: mol_type = other DNA; note = Bacterial
aaattcatttgag

SEQ ID NO: 29 - DNA, 13 bp, unidentified
  source 1..13: mol_type = other DNA; note = Bacterial
aaaatcatttgag

SEQ ID NO: 30 - DNA, 14 bp, unidentified
  source 1..14: mol_type = other DNA; note = Bacterial
aaaattcatttgag

SEQ ID NO: 31-37 - skipped (7 entries)

SEQ ID NO: 38 - DNA, 10 bp, unidentified
  source 1..10: mol_type = other DNA; note = Bacterial
gtttttgtac

SEQ ID NO: 39 - DNA, 11 bp, unidentified
  source 1..11: mol_type = other DNA; note = Bacterial
gtttttgtact

SEQ ID NO: 40 - DNA, 12 bp, unidentified
  source 1..12: mol_type = other DNA; note = Bacterial
gtttttgtactc

SEQ ID NO: 41 - DNA, 13 bp, unidentified
  source 1..13: mol_type = other DNA; note = Bacterial
gtttttgtactct

SEQ ID NO: 42 - DNA, 14 bp, unidentified
  source 1..14: mol_type = other DNA; note = Bacterial
gtttttgtactctc

SEQ ID NO: 43 - DNA, 15 bp, unidentified
  source 1..15: mol_type = other DNA; note = Bacterial
gtttttgtactctca

SEQ ID NO: 44 - DNA, 16 bp, unidentified
  source 1..16: mol_type = other DNA; note = Bacterial
gtttttgtactctcaa

SEQ ID NO: 45 - DNA, 63 bp, unidentified
  source 1..63: mol_type = other DNA; note = Bacterial
caaggacagttattgattttataatcactatgtgggtataaaaacgtcaaaatttcatttgag

SEQ ID NO: 46 - DNA, 103 bp, unidentified
  source 1..103: mol_type = other DNA; note = Bacterial
aaacaaagaattagctgatctttaataataaggaaatgttacattaaggttggtgggttgtttttatgggaaaaaatgctttaagaacaaatgtatacttaga

SEQ ID NO: 47 - protein, 1053 aa, unidentified
  source 1..1053: note = Bacterial
MKRNYILGLDIGITSVGYGIIDYETRDVIDAGVRLFKEANVENNEGRRSKRGARRLKRRRRHRIQRVKKLLFDYNLLTDHSELSGINPYEARVKGLSQKLSEEEFSAALLHLAKRRGVHNVNEVEEDTGNELSTKEQISRNSKALEEKYVAELQLERLKKDGEVRGSINRFKTSDYVKEAKQLLKVQKAYHQLDQSFIDTYIDLLETRRTYYEGPGEGSPFGWKDIKEWYEMLMGHCTYFPEELRSVKYAYNADLYNALNDLNNLVITRDENEKLEYYEKFQIIENVFKQKKKPTLKQIAKEILVNEEDIKGYRVTSTGKPEFTNLKVYHDIKDITARKEIIENAELLDQIAKILTIYQSSEDIQEELTNLNSELTQEEIEQISNLKGYTGTHNLSLKAINLILDELWHTNDNQIAIFNRLKLVPKKVDLSQQKEIPTTLVDDFILSPVVKRSFIQSIKVINAIIKKYGLPNDIIIELAREKNSKDAQKMINEMQKRNRQTNERIEEIIRTTGKENAKYLIEKIKLHDMQEGKCLYSLEAIPLEDLLNNPFNYEVDHIIPRSVSFDNSFNNKVLVKQEENSKKGNRTPFQYLSSSDSKISYETFKKHILNLAKGKGRISKTKKEYLLEERDINRFSVQKDFINRNLVDTRYATRGLMNLLRSYFRVNNLDVKVKSINGGFTSFLRRKWKFKKERNKGYKHHAEDALIIANADFIFKEWKKLDKAKKVMENQMFEEKQAESMPEIETEQEYKEIFITPHQIKHIKDFKDYKYSHRVDKKPNRELINDTLYSTRKDDKGNTLIVNNLNGLYDKDNDKLKKLINKSPEKLLMYHHDPQTYQKLKLIMEQYGDEKNPLYKYYEETGNYLTKYSKKDNGPVIKKIKYYGNKLNAHLDITDDYPNSRNKVVKLSLKPYRFDVYLDNGVYKFVTVKNLDVIKKENYYEVNSKCYEEAKKLKKISNQAEFIASFYNNDLIKINGELYRVIGVNNDLLNRIEVNMIDITYREYLENMNDKRPPRIIKTIASKTQSIKKYSTDILGNLYEVKSKKHPQIIKKG

SEQ ID NO: 48 - protein, 1368 aa, unidentified [sequence omitted]

SEQ ID NO: 49 - DNA, 56115 bp, unidentified
  source 1..56115: mol_type = other DNA; note = Bacterial
atgaaaatcaccattttagctgtagggaaactaaaagagaaatactggaagcaagccatagcagaatatgaaaaacgtttaggcccatacaccaagatagacatcatagaagttccagacgaaaaagcaccagaaaatatgagtgacaaagaaattgagcaagtaaaagaaaaagaagggcaacgaatactagccaaaattaaaccacaatccacagtcattacattagaaatacaaggaaagatgctatcttccgaaggattggcccaagaattgaatcaacgcatgacccaaggccaaagcgactttgtattcgtcattggcggatcaaacggcctgcacaaggacgtcttacaacgcagtaactactcactatcattcagcaaaatgacattcccacatcaaatgatgcgggttgtgttaattgagcaagtgtatagagcgtttaagattatgcgaggagaagcttatcataaataaaactaaaaattaagttgtgtataatttaaaaagttaatgagatgtggagggattacatatatgaaatattggattataccttgcaatatcatatgatgtttatagagtgtttaataaaggttctgttgcaaagttagaaaaatatagctaattactattttatcatgtcgttgttcccttaactggctaacatatgcctaatttcgtggcatggcgaaaatccgtagatctgaagagacctgcggttctttttatatagagcgtaaatacattcaataccttttaaagtattctttgccgtattgatactttgatatcttgtctttcttactttaatatgacggtgatcttgctcaatgaggttattcagatatttagatgtacaatgacagtcgggattcagtttaaacgctttaattactttagccattgctaccttcgttgaaggtgcctgatctgtaatcaccttttgaggtttaccaaattgtttaatgagacgtttgataaatacatatgctgaatgattatctcgttgcttacgcaaccaaatatctaatgtatgtccctctgcatcaatggcacgatataaatagctccattttccttttattttgatgtacgtctcatcaatacgccatttgtaataagcttttttatgctttttcttccaaatttgatacaaaattggggcatattcttgaacccaacggtagaccgttgaatgatgaacgtttacaccacgttcccttaatatttcagatatatcacgataactcaatgtatatcttagatagtagccaacggctacagtgataacatccttgttaaattgtttatatctgaaatagttcatacagaagactcctttttgttaaaattatactataaattcaactttgcaacagaaccgtattatggaatagagatgttggtaacatttatacaggatcattatacttaagtttaatttcgttattacagaaccacacattccaaccagaagagaaagtatgtctatttagttatggttcaggagcagtaggagaaatctttagtggttcaatcgttaaaggatatgacaaagcattagataaagagaaacacttaaatatgctagaatctagagagcaattatcagtcgaagaatacgaaacattctttaacagatttgataatcaagaatttgatttcgaacgtgaattgacacaagatccatattcaaaagtatacttatacagtatagaagaccatatcagaacatataagatagagaaataaactagtggccgattgtgcttgatgagcttgggacataaatcctaactcgaaataaataagcatatcactaaactgattttttaaagtttacagtgatatgcttatttttttatcttacgattttgtacgtgcatgcttgcctaggggtatggctcgagccctggagccattagtctctcgcacatactattccctcaggcgtcagcacttacaaaatcggttgtaattttcatttttatacgcattcttactgagattatactaataagaggaatagtaaaagcaattctaagtaaaattgcagataagaggtttgttaaaagcagttctaagtaaaattgcagataagaggtacgttaaaagcaattccatgcaaaattgctgataaggggtaagttaaaagcagttctcagtaaaattgcagataagaggtacgttaaaagcagttctaggcaaaattgcagataagaggtgcgttaaaagcagttctcagtaaaattgctgataaggggtaagttaaaagcaatcctaagtaaaattgcagataagaggtaagttaaaagcaatcctaagtaaaattgcagataaggggtacagaaaaactagacttgattacaaaatggagcttgggacataaatgattttttaaaaatgagatgagacgtagattaactccataatcaatacgaatctatcgacttctttatttatgatattcatctctttttaatggaaataaaagtgcgattaatgtgataatacagttacgttaattaaaaaaataaaaatgcaaggagaggtaatatgctaactgtatatggacatagaggattacctagtaaagctccggaaaatacaattgcatcatttaaagctgcttcagaagtagaaggtataaactggttggagttagatgttgcaattacaaaagatgaacaactgattatcattcatgatgattatttagaacggactacaaatatgtccggggaaataactgaattgaattatgatgaaattaaagatgcttctgcaggatcttggtttggtgaaaaattcaaagatgaacatttgccaactttcgatgatgtagtaaaaatagcaaatgaatataatatgaatttaaatgtagaattaaaaggtattactggaccgaatggactagcactttctaaaagtatggttaagcaagtggaagaacaattaacaaacttaaatcagaatcaagaagtgctcatttcaagctttaatgttgtgcttgttaaacttgcagaagaaatcatgccacaatataacagagcagttatattccatacaacttcgtttcgtgaagactggagaacacttttagattactgtaatgctaaaatagtaaacactgaagatgccaaacttactaaagcaaaagtaaaaatggtaaaagaagcgggttatgaattgaacgtatggactgtaaacaaaccagcacgtgcaaaccaacttgctaattggggagttgatggtatctttacagacaatgcagataaaatggtgcatttgtctcaatagaaagttagaggtgagtcttacgtttcagtgacggtagacttacctttaacatgttacatactaaaaaattaatttgaataagaaagagagacatatatgaaatacgatgattttatagtaggagaaacattcaaaacaaaaagccttcatattacagaagaagaaattatccaatttgcaacaacttttgatcctcaatatatgcatatagataaagaaaaagcagaacaaagtagatttaaaggtatcattgcatctggcatgcatacactttcaatatcatttaaattatgggtagaagaaggtaaatacggagaagaagttgtagcaggaacacaaatgaataacgttaaatttattaaacctgtatacccaggtaatacattgtacgttatcgctgaaattacaaataagaaatccataaaaaaagaaaatggactcgttacagtgtcactttcaacatacaatgaaaatgaagaaattgtatttaagggagaagtaacagcacttattaataattcataataaaacagtgaagcaaccatcgttacggattgcttcactgttttgttattcatctatatcgtattttttattaccgttctcatatagctcatcatacactttacctgagattttggcattgtagctagccattcctttatcttgtacatctttaacattaatagccatcatcatgtttggattatctttatcatatgatataaaccacccaatttgtctgcctgtttctccttgtttcattttgagttctgcagtaccggatttgccaattaagtttgcataagatctataaatatcttctttatgtgttttatttacgacttgttgcataccatcagttaatagattgatattttctttggaaataatatttttcttccaaactttgtttttcgtgtcttttaataagtgaggtgcgttaatattgccattattttctaatgcgctatagattgaaaggatctgtactgggttaatcagtatttcaccttgtccgtaacctgaatcagctaataatatttcattatctaaatttttgtttgaaatttgagcattataaaatggataatcacttggtatatcttcaccaacacctagttttttcatgcctttttcaaatttcttactgcctaattcgagtgctactctagcaaagaaaatgttatctgatgattctattgcttgttttaagtcgatattaccatttaccacttcatatcttgtaacgttgtaaccaccccaagatttatctttttgccaacctttaccatcgattttataacttgttttatcgtctaatgttttgttatttaacccaatcattgctgttaatattttttgagttgaacctggtgaagttgtaatctggaacttgttgagcagaggttcttttttatcttcggttaatttattatattcttcgttactcatgccatacataaatggatagacgtcatatgaaggtgtgcttacaagtgctaataattcacctgtttgagggtggatagcagtacctgagccataatcatttttcatgttgttataaatactcttttgaactttagcatcaatagttagttgaatatctttgccatcttttttctttttctctattaatgtatgtgcgattgtattgctattatcgtcaacgattgtgacacgatagccatcttcatgttggagctttttatcgtaaagtttttcgagtccctttttaccaataactgcatcatctttatagcctttatattctttttgttttaattcttcagagttaatgggaccaacataacctaatagatgtgaagtcgctttttctagaggatagttacgactttctgtttcattagttgtaagatgaaatttttttgcgaaatcacttaaatattcatccatttttttaacggttttaagtggaacgaaggtatcatcttgtacccaattttgatccatttgttgtttgatatagtcttcagaaatacttagttctttagcgattgctttataatcttttttagatacattctttggaacgatgcctatctcatatgctgttcctgtattggccaattccacattgtttcggtctaaaattttaccacgttctgattttaaattttcaatatgtatgctttggtctttctgcattcctggaataatgacgctatgatcccaatctaacttccacataccatcttctttaacaaaattaaattgaacgttgcgatcaatgttaccgtagtttgttttaattttatattgagcatctactcgttttttatttttagatactttttttattttacgatcctgaatgtttatatctttaacgcctaaactattatatatttttatcggacgttcagtcatttctacttcaccattatcgcttttagaaatataactgctatctttataaacttgtttgaaatttttatcttcaattgcatcaatagtattattaatttctttatcttttgaagcataaaaatatataccaaacccgacaactacaactattaaaataagtggaacaatttttatctttttcatcaatatcctccttatataagactacatttgtagtatattacaaatgtagtatttatgtcaaaataatgttataatttttgtgatatggaggtgtagaaggtgttatcatcttttttggttctgttgcaaagtaaggttctgttgcaaagtaaaaaatatagctaaccactaatttatcatgtcagtgttcgcttaacttgctagcatgatgctaatttcgtggcatggcgaaaatccgtagatctgaagagacctgcggttctttttatatagagcgtaaatacattcaataccttttaaagtattctttgctgtattgatactttgataccttgtctttcttactttaatatgacggtgatcttgctcaatgaggttattcagatatttcgatgtacaatggcagtcaggtttaagtttaaaagctttaattactttagccattgctaccttcgttgaaggtgcctgatctgtaattaccttttgaggtttaccaaattgtttaatgagacgtttgataaacgcatatgctgaatgattatctcgttgcttacgcaaccaaatatctaatgtatgtccctctgcatcaatggcacgatataaatagctccattttccttttattttgatgtacgtctcatcaatacgccatttgtaataagcttttttatgctttttcttccaaatttgatataaaattggggcatattcttgaacccaacggtagaccgttgaatgatgaacgtttacaccaagttcccttaatatttcagatatatcacgataactcaatgcatatcttagatagtagccaacggctacagtgataacatccttgttaaattgtttatatctgaaatagttcatacagaagactccttttggttaagattatactataaattcaactttgcaacagaacctcttaatcttattggatacaataactaacttaaacacattatctacaagtaaaaacttgtaaaaagaacatgtgttcttaattagtgtataattagtttaaattgattatggggtgatgtaatgaatgagagtaatcaaattatattcgatcatataacaaaggctattgaaaatatgaaaaataaaggctgggaaacaaggtatgggcaagaaactttaatgtatgatgtatttgatgcttatgattcaagagaaaatttaatagtagaagcgcaagtaggtataggaaaatcatttggatatttaattcctggtatattgatttcaaaaagtactaaaaaacctttaattgtaacgacttcctcaattcaattaactgagcaactagtcaatgatatacagcaagttgaagaaattttacatatatctgttgattgtatagtaggtaaaggtgtaactaactatccttgttttaaagaaattcatcgtaaaaatttaagtaaattaaatttaatggaggctttagatatagcaaataatggtttaacaaaacaaactgtacgtgagactaatttaaaatggaatcaaatatctaccaataattgtattatgagtaaatgtcactataaaaatgaatgcgcttattttaaaatgagaaataagttaaaagagggaaatagatatattagactcaatgaatataagccgaaagtcataatcgttaatcaagatatgttaatgatgaattttaaaaagttaacctttggaaaagagagtttaatctatgatgatccttgtatgctaatcgtagatgaagttcacaacttagaagagaaacaacgtgctaacatgactaaaactattaactctaaaactatgataaataaaataaaagaaggcgcaaaccgagttggtagtagatctcggtatttaaaaaatataaaaatgattgaagattggtttaatcttcaaaaggatagtgccaaaagtgagatatacaaaaatggtaattgtttatctactggacgagttgatataaaacctgttagtcatcatcaaatggccaaattaattagtatgacaaaggaaatagttgaagaattcgatgttaataatattgttgtatttaaacaatcttcgttagttagtaatgaacaattagaaatagctaataatctgttaacattatttaaaaatcttcaaaataacagcgacaaatatatattttggactgaaataactaagcaagaccaaattgatatttcattttgtcccaataatattgctgaaacacttagaaaaacagtttttagtacaagttacccagttgtatgtctttctgcaacaattactaataaaactaataatgaaaatagctatgagtacattaaagaaataattggttttaaaggctatgaggaagatattaagtataatgattttccgtacaaggaaagcaggctctacatacctccaaacttaccaaaatttgataaacgtgatgttaaatattatgaagaaataggtaaacatatttttgaattggcaagccaaaataagggaggcactttgatattgtttactgctaaagatgacattgacggtgtatataatgatttatcaaaaaggaaatttaataaaactatctatgtagatgatggtagtaaaagtcaaaatgaaattattgaatcatttaaaaaaactaaaggtgtaatattgggtacgggagtattttgggaaggaatagacttaaaaaatgaattattaacattattagttattgtcagattaccttttcctacgattgatccaattacaaaatataagattactaaattaaatgatagtaatgaagcagttatagttcctgaaatgataattaaactgaaacaaggtgtaggaagattagtaagaacaaagcaggataaaggtttattagtgttattagattcaagaatgaataaacccatttataagcataaagaagcagtattagatgcattaccaattaaaaatatgattcataaagatgaagtcaaagatttccttaataacatttaaagtaagtagtaatagttatccaatattttctagttgattctcttataatatgtccaattaagtgtagacgattcaagatgatattgagggaaggatgagaatgtgtcttttaggtagctcatttgatgataaccttaaacataatatttactttcatcctgctgaaaaaagaggttacagtttcaagccgatagaatacattgggctatataaagacaaagcaataaaagctatcggaaaagtagacaaagtaatagtgacggaaataaatgagagctcattatccttgaagacagtttatcctgtaggtactgagttatcgattgatgagtatgaaatagttaaaaataaaataatggtgcttgggaaagaaaagtggactaatctattgaacgaaccccattattattacttaattgaagattttatagagacagactacaagaaaacatctaaaggtggatcgatgggagttaagtattttaatgtgaatgaaattttgaatagggattgcttaaccaccgaacaaatcgctaaagaattatgtaataaagattgggaatgataaatagtgaatgaagctataatgcaataatgtatgtataacataatcaagtaatgaaattaatgataagggagtatggagtaaagaattgaattagtttgcatggtctatgtatcttaaaggtgttgaaggagatacaccgaagtatgcagtaccaattcttgaaacagactttagtgatttaccatctacacatacgacagtcggatcacttgatcggtttcgagataagacaatgagcattaacagaagcgggagtaactgttgaattccatttatatccagttagatactagagtttgaagtgataaatcttgattcggatgctgaaataagtaaaagagcagttactgaatataatataagtataagtatgccactagatattttaaggggtatttattcacttttataaaatcatctgctaagatagtgtggaagatttttataggagctgattataatgcgacatataaatatgtcatacatcatacgctatagtactctaactcaaagataagaagtacttagttatgaatagcattcatttcacaaagtacttcaacaaaaatggaggaatatgaaatgaataaaatagaagtgtataagtttgttaaagtaaagcagttagtatatcaattgattaagttatatcgtacaaacgatatgaattcccataaaacacaaaaagattttttactaaatgaaattaatgatatctttaaagaaaaagatattgatatctcggactttattacatcgattgacgatgtaaaattaactaagaaaaaagcagaacatcttttaaatgaattaaaagtgtacatccaagattttgaaataccttcatcaagtcaactggagaaaatttttcgtaaagtaaaaaaattaaagagaccagatataaatttaattgatacaaaagaaatttcatatttaggatggaatgataattcttctaaccgaaaatatatcgtttataaaaatttagatgataaattcgaaggtatatatggcgaaatttcaccaaataaagtaaaaggattctgtaaaatttgtaatcaggaatctgatacatcactctttctcaataaaactaaacataataagagtagtggaacatatactaaaaaaggagattacatttgttatgacagttttaaatgtaatcagaacctagatgatataaataatctttacgaatttattgttaaaataaaatagatccaaacagccctgatctttagaactaatgatcagggttgttatattttgtacctcactcttaatcgatacgctgagccttataataaataaagctaagattggttagtgtgtaactttatgcaatttgaaaagatataatgaaataagagagttttggtgatgatattaatatttaaatagatctatagacaattaatcgctgttgatttttaacaaatcaattcaatttagttatgttttgtgatggcatactaattaaaaaaagaagaactaggttttgtgccctagttcttctttttatttaattgttattcctatttcttaataagcgtaatgaattaagtatgacaagtatcgcagcgcctgtatcacttaatactgccaaccaaagtgttaatagcccaggaaatacaagaatgaatgcaatcaattttatgatgatagaaaaatatatgttttgcttaatgatatttttagcttttttacttatagaaatcgtacgtgttaattgatttatatcatctgacataagtacgacatcagctgtttccattgctgtatctgaaccaatacctcccattgcaatacctacgtcactttgtgctaaagcaggggcatcatttatgccgtctccaatcatagcgacacgatatcctttattttgcaaatcttttattgcagctaatttgtcaccaggcattaattcagcataaacttctttaatacctgaaagttgtgcgattttttgggcagtacctttattatctcctgttagcattatagtgtttttaatgtgagtaccatttaattgttgtattatttgcttgatatttgaacgtaatgggtctgcaatagtaatcaagccatgaatcatgctagaagatgcaataatgatgacggtaaaaccttcttgctcatatttgtttatttcttctttatagttgttaatttttttgttaatagactcaattaattttacgttaccagcataaacgtaactttcatttattttacctttgatgccttgaccaacgatattttcaaaatcagttacataagcttttttaacatttaattgcattgcgtaatctacgatagcgttgctaatagggtgggttgagtaggattccaaactcatagcaatatttagcaatgttgtttcattagcatctatagttttaatcgtatccacctttggacgaccttcagtcaaagtacctgttttatcaaaagccaacgcagataaagtacctagaccttctaaatggttaccacccttgataagtacgccattttttgctgcacttccaatcgcagtaacgatagctaccggtgttgaaatgacaagtgcacatggacatgcgataactagtaattcaagccctttatataaccattcgccccacgtacctaaagagaatagaggtggtatgaccatgactaataatgctaatacaaagacgataggtgtataaatttctgaaaatcgatctataaaagcttgcgtcggtgctttattttcttgtgcttcttcaaccatatgaatgattttagaaagcgttgtatcttctaccaatttagacacccggatgtataaagtaccattttcattgatagagcctgcatatacttcatcgttaatcgttttatcaacaggtatcgattcaccggtaataggtgcttggtttaaactggaacttccatcggtaattgttccatctaaagggacgcgatcacctggtttgataagtaagatttcaccaactcgtatatctgtcaaatctttagtagttgttccgttttctgttatgacatttgctgttgtggaagtaatatccattaatgattgtatagaattacgtgttttatctattgaaattgtttgcagcaaggttccaattgtaaataacaatacaacaatcgcaccttcaaaatattcaccaatgaatatagcgccaataacagctacggacatcaacacattcatatctaagcttttagatttaatggcataatatgcgcttttcaatggttttatgccactaacaataatggctatgatatacattaaatttgcaattaatactggcaatgttgtcagagttacaactaaaccaaggataagaaataatgttgaaatgataggttttctgaatactctccatttggaattactacttttttttgttggacttaatgttgcagaataaccgattttagaaacttctttttcaatatttttagttttattaccttcaaaaggttctgttgcaaagttgaatttatagtataattttaacaaaaaggagtcttctgtatgaactatttcagatataaacaatttaacaaggatgttatcactgtagccgttggctactatctaagatatacattgagttatcgtgatatatctgaaatattaagggaacgtggtgtaaacgttcatcattcaacggtctaccgttgggttcaagaatatgccccaattttgtatcaaatttggaagaaaaagcataaaaaagcttattacaaatggcgtattgatgagacgtacatcaaaataaaaggaaaatggagctatttatatcgtgccattgatgcagagggacatacattagatatttggttgcgtaagcaacgagataatcattcagcatatgcgtttatcaaacgtctcattaaacaatttggtaaacctcaaaaggtaattacagatcaggcaccttcaacgaaggtagcaatggctaaagtaattaaagcttttaaacttaaacctgactgtcattgtacatcgaaatatctgaataacctcattgagcaagatcaccgtcatattaaagtaagaaagacaaggtatcaaagtatcaatacagcaaagaatactttaaaaggtattgaatgtatttacgctctatataaaaagaaccgcaggtctcttcagatctacggattttcgccatgccacgaaattagcatcatgctagcaagttaagcgaacactgacatgataaattagtggttagctatatttttttactttgcaacagaaccctttttgcaataatacatttaattaaaaccttgttttaaacatcgatgacaagatctaatgtaggacgtggagacatcattttcggaatgatataaataaatccataaatggagataaatcgaaaacatttatacccatagggggtatgtgttatagtataagtatagctaatataatattttcataaataggaggggttaatttgaataataatggtgaagagcataatcctcaaaatcacatgaatcattccaatcacatgcatcatgataaccatgcctcacatcatcatagtggccatgcacatcatcatggaaattttaaagttaagttttttgtttcattaattttggcaatacctatcattcttttatcgccaatgatgggtgttaacttaccttttcaattcacatttccaggttctgaatgggtagtgttaatattaagtacaattttattcttttatggtggtaaaccgttcttgtctggtggtaaagatgaaattgctacaaaaaaaccaggcatgatgaccttagttgccctaggtatttcagtagcttatatttatagcttgtatgctttttatatgaataactttagtagtgcaactggtcatacaatggactttttttgggaattagcaaccttaattttaattatgctattaggacattggatagaaatgaatgctgtcggaaatgctggagatgctttaaagaaaatggcagaactgttacctaatagtgctattaaagttatggataatggccaacgcgaagaagttaaaatatcagacatcatgactgatgatatcgtcgaagtaaaagccggagaaagcattccgacagatggtattatcgttcaaggacaaacatctatagatgaatccctagtcactggagaatctaaaaaagtacaaaaaaatcaaaatgacaacgtcatcgggggttctattaatgggtctggaacaatacaagtcaaggttacagctgtgggagaagatggatatctttctcaagttatgggacttgttaatcaagcacaaaatgataaatctagtgctgaattgttatctgataaagtagcgggttatttattctactttgctgtaattgttggcgtgatttcttttattgtctggatgctcattcaaaatgatgttgattttgcattagaacgtcttgtaactgtgttagtcattgcttgtccacatgctttaggcttggcaatacctttagtcactgcacgttctacttcaattggtgcacataatggtttaattattaaaaatagagagtctgtagaaatagctcaacatatcgattatgtaatgatggataaaactggtactttaactgagggtaacttttctgtgaatcattatgagagctttaaaaatgatttgagtaatgatacaatattaagccttttcgcctcattagaaagtcaatctaatcacccattagctataagtattgttgattttgcgaaaagtaaaaatgtttcatttactaatccacaagacgttaataatattccaggtgtcggattagaaggtctaattgataataaaacatataaaataacaaatgtctcttatcttgataaacataaacttaattatgacgatgacttatttactaaattagctcaacaaggtaattcaatcagctatttaattgaggatcaacaagtcattggcatgattgctcaaggagatcaaattaaagaaagctcaaaacaaatggtagctgatttactatcaagaaatattacaccagtcatgcttacaggtgacaataatgaagtggcacacgctgtcgcaaaagaattaggtattagtgatgtccacgcacaactcatgccagaagataaggaaagcattataaaagattatcaaagtgacggtaataaagtcatgatggtcggagacggtatcaacgatgcgccgagtcttataagagccgatattggtatagcaattggtgcaggcacagatgttgcagtagattcaggtgatatcatacttgttaaaagtaatccatcagatattattcatttcttgaccctttcaaataatactatgagaaaaatggtgcaaaacttatggtggggtgcaggttataatattgttgctgtacctttagcagctggtattttagcgtttatcggcttgattttatcacctgcaataggtgctattttaatgtcgctaagtacggttattgttgcaattaatgcctttacattaaaattaaaataaaagataggagttttattatgattaaaaaattattttttatgatattaggatcattactaatattatcagcttgctccaataatgatgaaaaagataaagacactaatgaccaaaaaagtgagagccatatgaagcataatgatgaaagtaaagttcctgaaggtatgaaatcgactaatgagggtgaatttaaagtaggagataaagtaacgattacagcagggcatatgccaggtatgaaaggtgcagaagctactgtaaaaggtgcgtataaaacatatgcttatgttgtaagttataaacccacaaatggaaatgaaaaagtaaacaatcataaatgggtcgtaaacgaagagatcaaagatgcacctaaagatggatttagtaagggcgatactgttaaattagaagcaagtcatatgtctggtatgaaaggtgctacagtcaatatagataacgtgaaaaagactactgtttacgtagttgattacaaatccaaagataatggtaaaatcattaaaaatcataaatggatgacaggaaatgaactgaaagcacgataaaaatctagttctagattgagaaataaatagatataaagatatcctccttaatcaataatttaaataacttattattgttaaggaggatattttttagtgtgtaaattaaaaagaattttagaagaataacatttatcaaaaaactgttcattaccttattaaatgaaattatataattaaaaaccgcatcattaaccgatacgcagaagcgtaccacaaataaaactaaaaaatagattgtgaaaaatttatctttgaaaggggtcgaatgagagacatagaagtagaaaaagcctataagatgatgaaagaacaaggtaaaataaattttagtgaataccataagacactattacatatacatactctaggatcacatgatttaaaattatatgatgaatggaacaaacaatatttctatctattagccaagatgaaatatttagaattgctaaaaaagaaaatattctttacagtgagtattctaatataaatgatttaaaggaattagatatttttaagaactataaaaatctaaaggaaatgctttcttattttattttggtatacagcatatatactaatggaatatcaatagttgttgttgcagatcataatactgtgtgaagaatggaataaagaattctgtacggcttctgttctactcttttttattaaaaatatataataaagaattttttaaaatagtaaaatttatactttgattaacttttgacataattatgaacatctaaataagtaaaaatcaaatatttgaaattgtgttaatatgaatgtagaaactaaggtaataatttcatttaaaatagcttttaaaatttatatacatattagcgttgtgatacacgtagaaagggggaatcaaaagtggaaacgctaatggttaaagcaatggggacggtgatacgtttatcgattgaacatcaacattcgagtacattacttcaagaagctgaattaaaaattcatgattgggaatctcaatttagtgctaatgatccaaaatcagatttgatgaatgtgaatcaacatgcaggtatcgcaccagtcaaggttaatcctgagatgtttaacatgatacgttatggttatgaaactacactatcttctaattttaagatgaacatattgatagggccattagttaaattatggaaaattggtttcaaagatgcattgaaacctaaagaagaagatatacaacgcgctttaatgtgtatgaatcctgaaaatcttgttctaaattcaaagacacatgaagtatttcttacacgaccaggaatggagattgatttaggagccattgtaaaaggttattttgctgatcaattacagcaatactttttatctcatggtgtagcttctgccattatcgatttaggtggtaatgttttaacaattggtagacaaccggaaactctagaaaaatggcatgtaggtatacgcaatcctttttataaagatgcattatcactcgttacattaaatgtagagcatcaatcagttgttacttcaggcatctatgaacgctatttcatacaggaacatcaattatttcatcatattttggattccaatacagggtatcctgtagataatgatatcgctagcgtgacaatcatatctgatcatgggattgatggcgaggtatggagtacaatttgtagttttggtcaatcacaacaaaatattgaattattaaacctcatagatggtgttgaaggcatcattgtgacaagagatggaaacgttttaatgacttcaaaaatgcaaaggtatttataaaattttaaaaaatactcataaagagtattttatttttaagtataaatgtgaaaaaaatcacaatgtattaggaggaattgctatgagtaaagaattatttgatacttttaaatttaaatgtggtgccgaattaaaaaatagagtattaatggcgcccatgactatccaagctggatattttgatggaagtgttacatcagaaatgattgattattatcaatttagggctggtgatgcttcagcaattattgttgaaagttgttttgttgaaaaccatgggagaggcttcccaggagctataggtattgataacgatgacaaaatacctggacttaaacgtctagcagaagcgattcaatctaaggggtcaaaagcgattttacaactttatcatgctggaagaatggcgaatcctaagttcaatgaaggtgaacaacccatatctgcgagtcctattgcagcattaagacctgatgcggtaccaccaagagaaatgacacatgctcaaatcaatcagatgatagaagatttcggagaagcgacacgtcgtgctatagaagcaggatttgatggtgttgaaattcatggtgccaacacatacttattacaacaatttttctctccgcattctaatcgaagagaagatacatggggaggcagtcgtgaaaaacgtacgcgattcccaatcgaagtactaacaaaagttcaacatgtcgttgatgaaaatgaagcttctcaatttataataggatatcgattctcacctgaagaaattgaagagccaggcatacgttttgaagatacaatgtttttactaaatactttagcaaaatatgaacccgattacttccatatatcagcaaacagttatcaacgtacgtccatagtgaatcaagaagatacagaacctttaattaataaatatcataaaatgcaaagtgcacaattggcacaaattccattaatcggtgttggtagtattgcgcaacgaaaagatgcagaacatgcccttgaactcggttataatcttttaagtgttgggaaagcctatttagtagaacctcaatggacggataaaatttcacaaaacgaagaagttgaacaatttgtcgatatacatgaccaaaaaatacttcacataccatctcctctatggaaagtgatggacttcatgattttagataaagaagaagaacatcgtaaatatgaaagattaaaagcactacaaaataaaaaagtgaaatttaacaaaggcacgtatcatgtttatgcaaaaggtcataatggcaatctaccaatgaaagttcaattgtcggaagataaaattgtaagtattgaagtagatgatagtggagagtctgaaggtatagcgaacccagtttttgaacgtttacctcaagatatcatcaatggacaaacgttaaatgtcgatgtcatatcaggtgcgacagtaacaagtgaaggcatcgtacagggcattgcagatgcaattgaacaagcaggcgaagatccagatattttacgagcacgtcctaaaccagtcgttcagtggtctgatgaggtcgttgaagagacgactgacgtagtcgtgattggtacaggtggtgctggtttaagtgcagctgctacggttttagacgaaggaaaagaagtcatcatgcttgagaaatttgcggctataggtggcaataccatccgaacaggtggtcaagtcaatgctgctgagcctaaatggcaaagtgcattccctgcactcgctggtgaaaaagacacattgatacagttattaaatcatgatgaaaaggatatagatgaggcttatcttgaagatttcaatactttaaagcgtcaaattaaagattaccttgaaaaaagtagcaataaagatgattatcttttcgattctgttgaattacatcgcattcaaacgtatctaggtggaagacgtaaagatcgtaataatgtcgaaatttcaggtgattatgatttagttaaaacactcacagataatgttttggaatcagtatactggttgaaagataaaggggtacattttgatcgttcatttgtagatatgcctgttggtgcactatggcgtcgtggtcataaaccaatgaaagcacaaggtttagagtacattgaaaatctaggagactacgttaaacagcatcatggtcgtatttttacagaaactactgcagaaaaattaattaaagaaggtaatcaagttgttggtattgaagcacgtaaagcaaatggtgctaaagttaagattcacactcgtcacggcgtagtgttggccacaggtggttttggagcgaatactaaaatgatacaacaatataatacgtattgggataacattccagatgatattaaaacaacaaattctcctgcaattacaggtgatggtatacgtttaggtgtgcaagcaggcgctgacatcgtaggtatgggattctctcaaatgatgccgatttctgatcctaagacaggtgcattattcacaggattaatcgtgacaccttcaaacttcgtcttcattaataaggaaggccatcgttttgttaacgaatttgaaagtagagatgtattatctaaggcagcattagaacaaaaagacggcatcttctatattattgcagacgcaaatattaaagcgctagctatgaatacgactgaagacaaaataaatcaagaattagaagatggcactttaataaaagctgataccttagaagtgttagctcaaaaattaaacatagatgcaactacttttgtgaatacgattgaaagatataatactttcgtagaactaggacatgatgaagatttcaataaaaatgcatttgatttaaaaatcgaaaaagcaccattctatgcgacaccacgaaaacctgcaatacatcatactatgggtggtttgaaaatcaacatacatgcacaagtcgttgatgtagaaggtcatatcattaaaggattgtatgcagctggtgaagttgctggtggtatacatgcgggtaaccgtctaggtggtaatgcactggcagatattttcacttttggtcgcatcgctggtcaaagtgctgtaatgaaataaataaagaagaacaggaggacatttaatgatgagtgaacagtttaataaaggaaaacaactcattgtagcgattattttagggattctcacatattggttgtttgcacagtctttcttgaatatcgcaccacatgttcaacgtttctatgatgtagatatgagtattgttaacattgcggtcagtctcacatcactcttaactggtgtatttatagttgtagcaggaggtttatctgataagttaggtcgagttaaaattacttacgcaggtttgatacttagtatacttgggtctattgcactgattatatctcatgcgccacttttattattggtaggtcgagtgttacaaggtttatctgcagcatgcctacttccagcaactattgcgttaattaattcattctttcatggtgaagaaagacaaaaggcactaagttattggtcatttggttcatatggtggaacaggattagcatcactatttgctggaatgatagccacttttattgagtggcgttggattttcgtgttgtcaatcattttctcaattcttgccttaatattgcttaaaggcataccagaatctaaagatgaatctgcacataataaaaaatttgatattattggtattattatttttgtcattatgatgttaagtattaacatagtaataacccaaggtgatagaattggatggttaaatcctattattgtaatattaattgccatattcattgtgacattaatagctttctatatatttgaaaaacgtcaaaatgaacctttcatagattttagtttattttcaaataatatttatattggcacaacattagctaatttaatggtgaatatggatataggctcacttgcattatttaatatctatgttcaagatgataaacatttaacaggagcacaagcaggtttaattacaattccatatatgttgtgtagtttattaatgatacgtgtaggtgaacgttttatgcaaaatcgaggaccgcaattgccacttatgctaggtcctatatcaattacagtgggtattatacttttagccttcacttcgttgcctaacatgatttattatattgtagcgtgcatcggctttatctttataggtttaggattaggtttctttgcgacaccagcgctatctacagctgtatctaatgttccgtcagaaaaagcaggtactgcatcagggattatcaaaatgacttctacactcggtgcagcatttggtatcgctgttgtaactacaatctatacggcattgtccgtcaatcatccagcacaatttgcagctacaatcgcatttatcgtgggggcaggtttagtgtttatcgcatttattgccgcgtattgtttaattcctagaaagaatgtagatgcttaaatcgagagttggcgcagtaaatatcattgcttgaattttgatcgtatgttgaatgatgaataaatagttaaacttgatgatagtcttgaaataggagatgcgtttgaagccttttcttcagaattacgcttggaagatatcaatcaccatccgctgttgcaaacttagtatcattcttagcttctaatgattctgactatattactggtcaattcattttaactgatggtggattagtgtatagataaaaagggatacttcgtcatgataattaatggataaaaaaagcgtttaaatatttatatataatgattgtgtgcttatacaaaatgtcaactcaatgcattcatgtgagagtgggatgatgagtctgagacataaagtctctggataagtcaataaagacaatttctattgaaataatatagaaattgtcttttttataattttttgattattttcagattattgagctgctacttttcttatattgagtgccattaatacaaatccaagttctcttttaattttatttattcctctaatggatattcgaatgaaacccgttctagtaatttagttttgaacccacctaaatgaatatatgagttattttttatactataaaatatattcagatttcaatagtgacataaaataggcatctttatatttacctttagtgtagaattgctctttgagtaatccttcagttttaaatccttgtgattcgtatatatgcacagcttttttgttatctgtatcaacatatagataaattttgtgcatatttaatatatctaatgcataatttatcgctttttcgaatgcgaattttgcataacctttaccactgaactcaggtttaataattatttgtatttcacaattacgatggatgtaattaatttctactaattcaacaattcctatgacttgattttcatcttcaacaataaaacgtctctctgattcatctaataaatgcttatcaaataaatattgaagttccgttaaggattcataaggctcttcaaaccaataagacataatagaatattcattatttaattcatgaacaaaaagtaaatcactatactctaatgctcttagtttcataattccactcctaaaattttcctatatatttgcattataaatataaataacgaataagttatcattcactgtgaatactctattttaacaattcactacatactaattctcattttcttattattctctaatatctctgatttattactcttactatgaaacatataaaactgtcacatttgtttatattaataataaatacatcaatgataacaaaaagaaaataaaaaaataaaaatagagcatccctcaccgtaaaagtgaaggatgctttatttttattagaatatagttttcattttgatagataatggttaataattgtctataaatcattattaaggaccgttgtaatacaatcgtcattcataaaattttcatagattttatccaatattttttcatcttcaattgctgtgaaatgatatactagcccttttactattgatacatactttcttcttatgaggttttagcatttccatcacttgttcgacacgttctacaacaactggtcgcttcgcataagcaccataagctagaatcactgtgtcactttcgctaatcgctttcatcaagtgaatatcagtgtgctcatcgtatggatttttgatgtgtttgagattttctggacttttaatattagagaatagatttacaagatatacagcaccgtatctttctgaattagctaattggttgaggatgagaacagttgtgagatcgagtgataatacaccatctaaatgaggatacatcgttatcactgtacaaacaggtttcttttcatcccacgtctttttgagtaagtatcggtgtttttcatcgtcgctaaatatcgcttctgtgtatatcgtacttttgattgtattcatcatcttcactccttttagtattcttctggtaaaagcatcacataataaaaagtgtctacatcatcttcacgaatgacgtagactttcttaggtactgcattttgattttttacatagtttgtatagtgatattccaatttgtatgcgggctgttcttgttcatgagtaatagagagtatattattatcttcttgtagtttaaaaatgtgtaggtaatctgtatgaccttgttgatctctttcttttaccatattccaaagtaagatttgaaggtctagagatagttgttcactaatgcctcttgtgatgtatcgattgattttcatactattttcctccattttgcttttctttcatgatgtcaatcacttcgttaatgactgtaacagatatttatgccactttgatccaattattcatagttattccctccttctcttagtaaatgacgttcatcgataatcgtatttttagtatctgtgaggtatagaaagtccatatcaaaatgatccagataaccaatgctgatgagttggttattggcgtacattagaaatggatagatacttagctcatgtagctcattattatagtaggtataagtttcaagtatgagatgtgccagtggagaattattaataaaacgttccggtagaatattttctgctgcttcttctaacgcttcacattcccatgtttcgttgttagatagttggaatagatgagttatatattgtttgagttcttgagtgattgtttccatatcattgcctcctagatagtgtgatagtgatgtagttcatatacatcaatgggataatatatatttgatttgtcatttattacgaatcccggtaagaataagagaaaattccgatcaaaaacccgtgataaacgttggtgtaacaaggaaatcccggaatcccactcattttgacgaacaatcaactcattatttataagtattgatgatagggttgggtttctgcttccttatatatattatttatttataaagaataacgggattttgggattgtgcttgcacaatccttctgcttcttcgagtaagcaaatcccattcatttcccgttaaaaaatcatcgtgggatgttctttagcaatttcaatataagcttcgtgtagtagtagatagataatgcaatttgctaccatattagataagtgttattgaaattgataaagagaattcttataaatagttataaaaagtaatcagaagaagaaaataaagaactttctataataaaaagtcttcactattaaattttagtgaagactttttacttaaaattttattatttataaaactaagccaataatacttgctgaaataattgatgctaatgttgcacctaataataatcttagggcaaaagaagctactttatttccctgtttactatcaatacctttaatagctcctaccataattccaacagtaccaaagttagcaaagcttacaagataaacagatattataccttgagtctttggagatagagaagaggcaattttttgaaaatctaacattgctacgaactcatttgtaattaactttgttgccataattgatccagcacgtatagcttcactccatggaatacccataatgaaagcgataggagcaaatatgtaaccaatcaattttttaaaatctagaccgactaaatcaaatacaatagtaattcctttcattaaagatataaaagctaacaacattattgctacagtaatagcaattctgaagccatcaatagcactttcaccaatcatttgaaagaaagttgtttttttaatatttttttctgattcagcttctaattctttattatcatttttgtaaggattaatgacgctagcaattatcaaagcactgaaaatatttaaaacaactgcagtaactacatatttaggatcgatcatttgcatatatgagcctagcatagccatactgacagcactcatacctgaagtagcgatagtatataacttttcttttgacaagcttggaataatatttttaactgttaaataaacctctggttgacctaacatagaagtagatattgcgatatagctttcaagttggcccatatgagttattttattaattatccaacctataattttaattagaaaaggtaaaattttaaaatagtttaacataccaattaaaactgaaataaaaactaaaggtagtaatacatttagaaagaaattatagccgtttttattttgtaaatctccaaaaacgaattcaataccttctttactaatattcattaaaccttcaaaaaatgtactcattgcggttaataaattaagacctattgatgtattcatcataaataaaacaagaacaatttgtattactatcataatcattggtttttttatatctatagcttttctattaaaactaaaaatatatgcaactaataaagcaaaaactattcctaaaaatgtgaagattattgacatagtcaagcacctacattttgctgaaagctacagctattttagctcctaaaacagcgttattttctaccaacttaatatttgtttctaagcttttgccatctgttttttcaacgattgttttaagaaggaaaggtgtagagtcttttccactaattccattggcaatagaatctttaacagcttcttcaattatagtgtcaatataatctttagaaagttcatgttctttaggaacaggatttgcaatgaccattccaccatgtaaatttaactccattttggtcttgaaaatttcagctatttctgtaggttcctcaactgaactatttagttttaaaccgctttctctagtgaaaaaagcaggtagttcagttgtttgatatccaattaccggaacacctttagtttctaagtattcaagcgttttaggcaaatctaaaatagattttgctcctgcgcatataactgtaacatttgtatgcgctagttcttctaaatctgctgaaatatccatactagtttctacgcccttatgaacaccaccaattccaccagtgacaaaaaatggtatcccagctaattctgaacaaatcatagtagaagcaacagttgtagccccaatttttttagtagcaactatttctgctaagtcgcgacgagatactttagcgacattaggactatttgctagagtctccaagtcattttcgtttaaaccaatttttattttcccatccattatggcaatagtagcaggtgtggcgccattgtctcgtattatttgttcaactttttttgccatttcaatgttttgtgggtagggcataccatgagagattattgtagattctaaagctactatgggactattgttttttttggcttcttcaacttctgtagaaaattcaagaaattttttcatttttaaattcctccaattcaatttctaattgtttttgatctaaattttgtctaacagtgtaattagtttcaacagttttcttcgagtttaacaaagctaagttaataatgtcttcattagtataattttttagccaactatatattactgcgctagtaaatgaatcaccagcaccagttacatcaactacatttttagatgaaattactgagtgaaatgattctgaactattatctttgaaaatgagtggttttagtccatttgtaataatgacgttagacacaccaagattaattaatttctcagcagcaatactcatgtcatcattactatcaattttcatttttaaaaaagtttcagtttcatcgcgattaataattaaccaatcaattgaatgtagtgaattaggcatatggatcattttaggtgaagatactggtacaattactaacttaatattgtttttttctgcgaatgaagtgaggtactcaatagattttttgggtaaatttaaatctattactaaacatttagcttttaataagatagatgactgctttgacagaaattcaggtgtaatttcctcgtaaatattcatatctgcaaaaccatactgcatatcaccttttttatctataatagctgtatatgatcctgtacttgcattttctataggttgaatataatttgtattcataaaaggctcagatagttttttaatcaaactccattcgctatcatttccagctgctgttaaaaatgtaacattttcaccaagtctccctaagttttcagcaatatttcttgctacacctccaatcgattttgttgattttactggattggaagtcatagattgtagatcagtatcacaataaaactttctatcaacattagcagctccaatacagattatggaatcttcctcattaacaatgtatgcttttcctaatatatatttcttttttattaaaccagatattatattagctgtggctggccttgataaaccaatacgttctgctaactcttgttgagtaataaaaggattttttttaatttcgtttaaaataaattgctctttatttttcaaaatagcacctccttttaaagaaacaatagttcacaaacaaaacatttgtttgtttcattcaaagagataataacatatatacatttttgtgtaaacgttttcttgaagggttttattttttattctattaaaagataattatactcactttatttactaaataataagatacagtgtttgggacaaaaataagaggctgggacaaaataaaatgtctcagcctattttatcattttgtcagtagctgactgatttgaaaatgcgcttgaatcaagcttttttcaaacctagtcatccttgctggggtaggacaacgaaataaattttgagaaaatattatttctgtcccactcccaagtggatggttattaaatagttgtttgataatctcattattcagtttgagcgtaacgtaaaattgcttcttatgatgctcatcttttcttatgtcaatacgatcgatgattgttagatatagtgatttcaactgagatttctctaatttgtctatatctttgaatattgcttgtaatacattagcaatcatatctgcatcataatgtggagattccgcttgtttatcttgttctagttgatggatttgattatttatttgattcaattcatcttggtagctaagtattgttggtttcaatacgctatctaagtcaggggagtcttcgatagttttcgttagtgtatgcattttggcttttatttcttcacattgtgactgtttataggcaatatcatgattcaaagaagatacgtctatttgacttctttcatttaccttttcaaccaattgcttcaatacctttttgcttttgataatttccaatatctgatccataacatatttttctagtacatctgctctaacactattggctgaacaaacttttgaacctttgtttctaaaattactacatgagtaatatctgattcttttcttagtgccatcttttaatgtattggtcgtattacttgcggccattgctgcaccacatttcggacattttacaatgccagtcagtaggttagtccctttaccgtgaacttgtggtttcttgcgactctcttggcgtttaaactgtactttatcccgtaaagctttatcaataataggcgcatgcttaccatctgcaatgattggttcttcattgagtccttttcgttttttatcgctccagtgtctatacttcgcaaactgtatctttccaatgtaaaaagggtttgagatgatgtaagtaatggacgaaatgctaaaaggtttcgctttcttagtcacataacctttatgattcaatgcgttcgcaatcttacgataaccatgacctttagcgtatgactcaaaaatatatttaacaatattcgcttcatgttgattgatcatgagctcttttttactgtcaggtactttatcatagcctaaaggtaaattaccttggtaataaccttcaatcgctcgttgtctttgaccgttataaacgttttctataatcgtatttctttcaaattctgcgaagctggctaaaatttggagcatcaatttacctgttgagctggcaatttctattttttcagttagactaaaaaattcgacattgattttatacaatttttccacaatatttaataagtctgaggtatttctagctaaacgattggttttgtagaccataatacagtctaacttaccgtcatttgcatcttttaacatacgttgtaattctggacgttccattgttttacccgatataccacgatcggtatattcatcaacgacctcataaccttgaaattgacaatactctgtaagttggtttaattgaccttgaatactgtaaccatttttttgagtttcagtcgatacacgggcatataatccaatatgtttctttttaagttgtttcatattacttccatcctttcagatattattaaatgtgattgttcaacgatattgagtggactatttttaaagtagataccttgtaattgtttagtttgagttattgtaatgtcattaatcaaaggtgctatggtttctaatgtcaatttatctttgattatatgacggattgtttcggtaatttgtttatgtgaataattagagtaacgttcttctctttcaaagccagcagataaacgtttaaacgtttcgatatcaatttgattttgtgccagtttttcgatgagttgttcttgtgttaaatgtgattgtctgtgtttcatttgttggtgttttagagcttttagtattgtcttatttaatttgtcatgaaatgacggattatcacaatatgctttacaagtgttgaggacctctgtttcaatcatttgcgcattgatacctttaaatggacacgtatgataggcttcattcatattcttaggacaaacatagtaacgtagggagtgtttctctttttttatcgttaagtttgttaatgttgattgacagtaaggacatttgattcgtcgctttagcttatttctagaattggatcgattgtgttgcttatgaatacgacgctcttgtgcttcttcaaacatatcaacatcaataataggcggaacgatatcattaaatgtgccatatttattaatgacacgaccgcaatagttaggattcaagagaatatttctaacttgatagggcttacgaggaataagcttaggatggttatctaaatgttgggaaatctttttgtagcctagaccgtgtaagtaccagcgataaactgctttgactgtataggcttcttcttcatgtacaacaaaatgaccttgtctataacgatacccaaaaggtgcatgagttgtgattagcttaccttgtttggctttttctcttgtcccatttcgtgtctgttcactgatattattagactccatttcagctagactcatgagtatgtttaagcgaaagcaatcaaacttttaagacaaatcaaaatatccatcgttaacactgatgattgtgacgtgatgctttttacaaatttcaaagaattgtatggcatttttcaaattacgatggagccgatttaagcgatagcaacataatactttacattttccagatgtaatcatttctaccattttttgataacccgaatgttttgtatgtcgacctgttttcttatcatcataaaatgttacattggaccatccatattgcttagcagtgtctataatgagggatttctgagtcgctaagctttgttgtttgagtgtactttgacgtacataagcaataacttcttccatgttatacacctccaaaaagataatatatatttgtgagtaaattcaaataaaggtccaacgtgcttctaacacgttggaccgcaatgattaataatcatgattttatttttcaataaagtaattagttagtgatgtaataagtttatatttcaaatatgaattatttaataaatattgtaaaatttcattaagttatttatgataaatataaattaaaacgttatttttattttatagtgaaaggattaataataatgaaacacatgcatttatctgttttagcttatagtacaggtctacatcctgcctcttggagactaccacattcatatgttgaagaagttggagatattgattttcaaattaagttagcgaaattagccgaaaaaggtaaactggatgcattcttcttaggtgatggtcaatatatttctggagaagaaacaggacatatttcttattattttgaaccactaacggcgcttgctgccatttcacgtgaaacacattcaattggtttgataggtaccatgtcttcttctttttatgaaccttatcttgcagcacgtatgctttcaagtttacatcaaatatctcatgggcgtattggggcaaatattgtaacatctcaatttgatttagaagcacaaaactactcgatgcaagctttaccacatcttgaaaaacgttatgaacgagcagatgagtttattaatgtaatgaaaaaattatgggaatcatttactgtagaggctatcgttaatcacaaaaactcaggaattggcttaaatcatcagtatattcatccacttcattatcaaggaaagtattttcaagttgccggagctattaacattccaacacccaaatatggtcgaccacgtttatttcaagcaggaacttccattccaggtcgtgatttagcagtacgacacgtggatgctattttttcaattgcatggaatttacaagatggccaacagttcagacaagacattcatcaacgtgccatggaagcaaatcgtcaaccccctcttgtattaccaggtctcactgtttatgttgatgagaatgaagaggatgcttataaacttaagcaacaattagatgatatgattccacttgaaaaacgcaagaaacaattatctaaagctattggtctagatataagtgaatggaaactagatgaagttataccgtccttaccagattatgaaacattatcgaaaaaggtcgtaaaatcagtatatgaagccatacaacgtgccattaagactgagcatcttacattaagagatttattagatcgttttggtacttgggtagggcacaagacaatagtaggaactcccgaacaagtggcggatgaaatgatcgaatggtttaaaaaagaagcgtgcgatggttttatgttgatggccccgacgtatccagaatcatttgaaaaatttattcatttagtgataccaattcttcaagaacgtggagtgtttagaagagattatgagagtcatctgttaaaaaatcatttgggtataaaaaactaaaaataaaccgcatcattaaccgatacgcagaagcttatcacaaataaaactaaaaaattggtaagtagatgaagagtgtaaatcagagtaattaataataatgtatcaaatttaaacaaaggggtctttaagtatgaatttaagaggtcatgaaaataggcttaaatttcttgagaaatatgatgtgacacctatatcacatttaaaattattagaagatcaaaagaaagacggtgaaggtggcatactgacagatagctattactgtttttcatacagcttaaaaggtaattctaaaaaagttttaggtacgtttaattgtggttatcatattgctgaagacttactaaaattatcaaatcaagacaaattacctttgtttaacccgtttaaagtaattaatgaaggtaatcaattgcaggaagtagcgaataaaggtaatttagatattaataggcaaagaaaacagtataatgaagtagctttacagctttcaaatgctataaatttaatcatattttgttatgagggtaatattaaagaaccactttcaacaataaaacacgaaaccgataaatattattatagtaaaccatatgatcgtaaaattaaagcagtaaatactattatcggtaatttgtttgataagaaattagttgagaaaatatctgaaattaatggaaatcaggaaattagaaaatttgatttttcattactcactgatgtaattaaaaaacacgagatacaaaataattttgaataataagtggatgtaagaagatattaaatattgaagctagtattaaggatattcaaaatattataaattattttactgaatgtggcgtgaataataagtattatgagagtgagaaaagaagtagtctaggaaagttggtaagtgttattggacacgaagaaaatgttagaaatccaaaataacctgaattagattttgaagatttcatatctgaatgtataagtgaaaaacaaaaaagaattagacataaactaggaggcagagtatgatgtcatcgaatgagatagtaaaaaaattatattcaaaggaagatattcgcatagaattagagctcactccacataagtttaaaaaaagaatggaaaccattactaagctttttaaaattgatatgaaaatttttcacaattacaaaggccaagataaaaataatcaatacacatttaatggcgtcgcaaaagaattaataaaggtgctactaaaaagtattgactattacccagtggatataaattccaaagcttttaaacaaaacggaaaatctaaaaaagagatgattgaaaatataaaagcatctagttacatggaatatacttatcagttaatgaaatctatcaatgaaattaaatacaaaagattaattgcagacatacatacgaaagacgtatatcaaaatactaaagcatggttaagtattggtgaatcaattaataaaaaggaacaagaattataccaatatatgacacctttgcccatacataaaagaattgagctacaaaatgaagtattaaaatctatagatgaaacgatttttcaatttatggcaaaagaacgtagaaacacccaaataaaagaaaataatgaattagaagaatacacaaatgcaataaaagaaggtaagtatcccaaaaaggattacgaattaaaccacctattatacgagaaaaatgaaatgccattagatagcttaattaaagatgtatgggactatgatgaaacagagtatatggagcttgattggttaattgcagatatgctaaaacgttcacaaagagctgatagtaattttatcgaaagtttagataagaaaaacaaattgagaaaaaatattcataaagaatctattaaaagtatatctaagttgattgatcatgaattggttaaaaataatagaaagtgggacgtagcagaattttataagaatcaacaattttggaacaatagtacattaagacgtagctctcaaaattttgggattttatattacaaaaaaaataggttacatacaatgaaccaaagtaatattattaaaaaaataaaaattatcgaggctaatatagagagtgcaaataaacagccgagctatttagatttctttttacaagctaagtttgacttagagaggttagaaagtgaattaatgaaatatagcattaatccgaaatattttaataagataaatagtgattacgtaagatatgctattgaagatgtacataatgcaattattaaaattgacagatatataagtaacgataaagtgaagttaaactattcaaatgcccaaatggtagtgagaaacgaaataacagaacaaggaagctactttgtaaaccaggcattgaatacactgtcaaaggtagaagagtctggctacagctttgataatttcatggtaggacctttcgtagaagactttaaaaaagcaattaaaaatcgtagatttggttctaaaacagattaagattgttttttagagttaaacataagaataaatttaaataaaaaaacaaacccaacaaaccttgttatatcaacgtttgttgggtttatttttttggtgattttttaataactcaattacaccttagtataatattgctaaattatacattgtcgaggccaagacaaataaaaaattaaagcaaaagttagcgcgcaactttctgccataaaggagcagatttatatggagacaagagacaaactgatgtcattgactcaaagtgacaaaacacaacaatggttaatgaacaaatcatctaaccaaactgatgttcaacaattgcagcaacaattcagtcagcagcttgaccaacaatataatgcacttttagctgatgaacaagctaaattagatcaatatgtggaagtccatcatgaattggaagcattaaaggaagaaattgaagcagaacctattacacttaatattgataaattacccgatatcaaagcgataatgcttgaaaaggctaagaacaatgaacattctgataaaatcgaacagttatttgatagattagatcagtcattaaatggtacgaatcgattatatacacaattatcgttgattggtacacgaacacatcgaatcacaactaaaaattttaatattcagggcttacctaaagcagtccaatgcacgattttaccttcaaaatataagaaggtatatactgtcgattttaaatcatttgaaccttcggttgttgcgtacatgactcaagattcaaaactgattgactttttaaatcagaaagacggattgtatgacgcattgctaagtgaattaggcttatcatatgagctacgagtatttgttaaacgtgcatttattggttcgtttctatttggtggcaacttcgatagcgctaaattcaagttgaaacaatatgtaagtgaagtgcaatggttggatgcggtcagccaatttacaaaagtcattgaacttaagaaacaaatcgaagagcataaaaccattcctatgccttatggcattgaacatgatatgagcgcatttcaaggtagcagtattatagcattttatgtacaaactgtagcgagttatgttttcaagcatattctgttggaagtgtacaaagcacaatgcgaacaaaaaacgtttaaaattattgtacctatacatgatgcgattatgattgaatgtgatgatgaagaaacggcgcaaaatgtatcgcagctaatgaaaagtaaggcaaatgaattgtttaatggtgagtttgcacacgtgacagtggaagcattagggggtgtaaacaatgaataatgatagaggaaaaagtttacaaattccaaaaagcatagccctaactgaaggatatatatatgttgcttcattatattctgtaacccaaacagatttcaatggggatgttaaacatcagtttacgtatgaaatagaggtagatcagaaagttatttatgtaaatcgtagtatttcgaaagatgctaccgataagcagttgtcaatcaatgattggcttaaacatcacagtaattatagctccactcataagaattatgccccctacattgatagaaagcatttaatccatgtaggttgctttaacggtaattattatgtacaagatgtagcatcattaaatgaagatggaggattattataatgaaacatatattcgatatgttaacaaaaataataagtgtggctaaggaggcagtcgaccgtcaaggtctgattgctatcctaaccatgagtattggcaatgatgatgaaatagaagaaacggtacaaggtgaaacagtgtataacgaacttatcgatcagttacgacttaatatcccaaaagatacggattatcgacctaacatctatagctatttcggtattaagaagaaaccaagtgacacaatattaatagacatgatgataaaagtttttcatatcaaacgcttcaattcggaactgtatatattcaaaattaacggttggcaaaagctaagtgaagacgagttaaaaggatttgtatcaaaaatgatacaagtactgttaatcggttatacgcctacgcaaagtgcactgaataatgtggttgaaggtctgcaaaaatcaacagatgtagaagaacttgtcgagaacgagcactatattggttgtggtgaaaatatgttcgatcttaatacattcaaagtcgttaaaaattcaatcgacatttttccaaaaacgcgattaaatttagcgttagataaaaatgatgagattactgaccagatacccaaacatttcaatcaatatatgttagaacttgcaaattatgacgatgatttacaatactttctttttcaacatacagcagtgttattgacggctgatactaaataccgtcgaggtctcatattatatggtggagctaagaatgggaaatctgtatatattgaactagttaaatcatttttctatagcaaagatattgtgtctaagccacttaatgagcttgaaggtcgctttgacaaagaaagtttaattgacaaaagtctaatggcaagtcatgaaatagggcaatctaggattcaagaacagattgtaaatgacttcaaaaagttattatctgtagaatcaatgcatgttgatcgtaaaggaaaaactcaagtggaagtcactttggatttgaaacttatttttagtacaaatgcggtacttaattttcctcctgaacatgcgaaagctttggagcgtcgaattaatattattccatgtgagtattatgttgaaaaagcggacacttcattgattgataagctccagagtgagaagaaagaaatctttctttacttgatgtatgtgtatcaacagattgtaaaagcagatatcgagtaccttgaaaatagtcgtgtcactgaaattactcacgattggttaaattttggatatgaatttgtttctagcaggtccgcaagtattgcaaatcagaaagagtgtattaatttactcagaaaacttatagaaatcaaaccaggatcacgaatcaaagtatccgagttaaataaagttattaatgaagaaataaaggtgagttctcaggttattaaacagttaattcaagaaaactttgatactcaaaccaaactatacaatggctacgattattggattgatttaggttggaaagaagccgataaaaaagagattcatgatatttcgaaaaaagataatattatttcattagaaaaaaatgaaaatataacagacgatgaggcattagatgaagagaatttggactttgattgggaggactttgacgatgaataatgaacaaattgaagcatttgtagaagtacttgtgcctatcatagaagaacgtatcaataaaggtaagtaatctaattacgtactacaggcagttgcctgtagtactcatatgattaagtgggaaaagtgataaaaatgaaacgaaattataaatatatattatccatatgatgttacaagaccgatggtctgtagcaataatctaataaaaggagcggtatgatatgaagggtaaaattgcactttattcacgcgttagtacgtcagagcagtcggagcatgggtactcaatccatgagcaagaacaagtactcatcaaagaggttgtgaaaaactatccaggttatgactatgaaacttatatcgattctggtatatcaggtaaaaatattgaaggtcgaccagcaatgaaacgtctattacaagatgttaaggataataaaatcgaaatggtgttaagttggaaattgaatcgtatctcacgatcaatgagagacgtgtttaatattattcatgaattcaaagaacatggcgtagggtataaatcgatttctgagaatattgatacatccaatgcttctggtgaagttttagttacaatgtttgggttaataggatctatagaacgccagactttgatttccaatgtgaaactttctatgaatgctaaggcacggagcggagaggcaatcaccggtcgtgttttaggctacaaattatcacttaatccattgacacagaaaaatgatttagttattgatgaaaatgaagctaatattgtacgtgaaattttcgatttatatttgaatcataataaaggacttaaagcaatcacgacaattctaaatcaaaaaggatatcgcaccattaatcaaaaaccattttcagtgttcggcgtgaaatatattttgaataatccagtctataaaggttttgttagatttaataaccatcaaaactgggcagttcagcgaagaggtggtaaaagtgatgaaaatgatgtgatattggtcaaaggtaagcatgaagccattataagtgaagatgtatttgatcaagttcatgagaaactagcttctaaaagttttaaaccgggtcgacctattggtggagatttctacttacgtggtcttattaaatgcccagaatgcggaaataatatggtatgtcgacggacttattataaaacgaaaaagtcaaaagaacggacaatcaaacgctattacatttgttcattatttaaccgttctgggagttctgcttgtcatagtaattccatcaatgctgaagtcgtcgagcgtgtaattaatgttcatttgaatcgtattctgtctcaaccagatattatcaagcagattgcgtcaaatgtgatcgaagaactgaaacaaaagcatagtaaccaaacagaaattaaatatgacattgatagtttagaaaaacaaaaagctaagcttaaaacacaacaagaacgattattagatttatatttggatgaggaaatagatagcgaaatattgaaagataaacaaagtcaaatgaatcaacagttagaagtattagatcaacaaattaaagaagcgcaacaagcaaatcaatcacaggatgaaatacccaattttgataaattaaaaggacgactcattttgatgataacacgattcagcgtgtacttaagagaggctacacccgaatctaaaaatcaacttatgaaaatgttaattgattcaattgaaattacgacagataaacaagtaaaacttgtaaggtataaaattgacgaaagtcttatcccgcaatccattaaaaaggattgtgggaatttttttatgcctaaatttaactttgtgataaatgtcacaaataaaaataggattgaaaatttatcacttttaccacttttttagagtgacaaaagtggaggagttttgaaatattttataaatatatattttatttatggagtacacattattaattaaggaggtcattatagtgacgctaagcaaacaacttaaaacgtatattactgaacgatttaaattaaattatcaagaaacttggagttgtgaaaccgtagacgcggtggctgaagacgtattacctgaaaaatatattaaaaatagtccactcgaacataaaatattgaacacatttacttattataacgatgaattacatgaaatcagtatttatcctttcttatactatttagataaggaattaatagcaataggttatttagataattttgatttagactttatatttttaaatgacactcatcaaattattattgatgaacgctacttgttacaaaaagggggcgagtaattatgaactggattaaggttgctcaactatctgttacagtcattaacgaagtgattgagatcatgaaagaaaagcagaatggaggaaaatagtatgaacatcaatcgatacatcacaagaggcattagtgaacaactatctctagaccttcaaatcttactttggcacatggtagaagaaaaagataaccagcctcataccgattacctacacattttcaaactacaagatgatgataatatgttgtcaattacacatgaacaagaacagcccgtatacaagttagaatatcactatacaaactatgaaaaaaatcaaaatgcattacctaagaaagtctacgtcattcgtgaagatgatgtagacgttttttattatgtgatgcttttaccagaagaatactaaaaggagtgacgttgatgaatacaatcaaaagtacgatacacacagaagctatatttagcgatgatgaacaacaccgctacttactcaaaaagacgtgggatgaaaagaaacctgtttgtacagtgataacgatgtatcctcatttagatggcgtattatcactcgatcttactactgttcttatcctcaaccaattagcgaattctgaacaatatggcgctgtatatctagtgaatctattctctaatattaaaacaccagagaatcttaaacatattaaagaaccttatgataaacacacagacatccatttgatgaaagcaattagtgagagtgatacagtgattctagcttatggtgcttatgcgaagcgacccgttgtcgtcgaacgtgttgagcaagtaatggaaatgttaaaatctcataaaaagaaagtcaaaaaactcataaacccagcaacgaatgacattatgcatccgcttaatcctaaagcacgtcaaaaatggacattgaaataaaggaggattatatatgaaccataacactacacaatcagattggcgaatagttgctagttgcttagcatcacaaaattatatatctatcgtaaaaggattagtacatcattttacagcgattgcagatgaggaaacacttgataaaatctatgaagattttatgaatgatgactctataaccacggtacttaataatgatttacagacaattattaaccattatctgtcaaaatgaaaattatattctaataaaactagagcatccttcacttagtggtgagggatgctcttatctttatttttttgattaatattttactcaggaaattttacattaaatttaaaagtattatacaattaaattattagtttctagtgaagaaatacgtattaaatttattattaactgtagcacattatcaagcaattgtactgttaaaagggattggtcattcaatgagacaatatgtttatcaaaatgatattaatttaataaactctttatatgagagtgatttttggaagataataaaagaagacgcagcatattatcataaaaataataaattcaagaaagataatgctatacgaatacttgaatctctaattaaatcaatatatgtagatcctgatggttttgataaagctcttgcagctgaaatgcaagatttctataacaaaatgcaaaaatcacaatacatcaaagagtcttattatcttagtattaatcaccagaaatgtagtctagatgctctcatcggatggaaaccacttttccgatttagaaatggtgataaaaaatggttagatgacttagaacttattagagggaatagaatgggccatttagcttttccagtacaaaaaaattctcttaatcaactaagaggaattttattaaaagatagaattgattatactctatttgatattaaattattttatgaaaatgcagctcatttaaaattacagaaagcttatgaacaagaaccaacacgaaaatggctaaaatcatttggtacctttaatcaatttatagagcgtatgcaattgaactacttcgtctataaagatccaatcacattaaaatatgatgttattgacttatcattgccatataataatgataagtcacattgcttaaaagaaattccaaaaaaaattaaggtcgaagaaacttatattacaaatatacttaattatattaaaaaatatggcgaaaaattatctactatccatgtggacttaatgattgattatcatgtataaataaaagaacaacccttcaccgtaaagtgaagggtgctctttagcttctttcattatttacaaatttcatctctttttttgatacaattctaacttaattaaatataatgctactctataaatctcctacatatttatagctcatatcctctaaaataaccagtgagtatctatacatatattttatggtaacgtaggctttttctagtttacattttattgattactcgctataagttctgtttgctcgacaacttgttcgacagtcatcttttgtaaatcaggaggataaccatattttttaagcaatcgtctaaaagttaagcgcatttttacttttgcactatcgcgtttagataaattgacgcccatattttttcactgttttagttagctcatgagcaattgcacgtagttctttatcaccattgcctctttagttatttcatgtgatgaagctaatgcataataaaatacaaggtccttaattactattgagatgttagaaaatattaaagaaagcaatttttactaaattttaaggacattacgtttttataattaaattaaagttagcttttataagaaagatattcatacttaataaaaaaaaactattaaattttgtttgactaaagttggatagtacattatagtataattacaatactaatgtgtattgtacttatacctaaaattacagaatctactaaaacaaggcaaaatgccgtgtttatctcgtcaacttgttggcgagatttttttatatcaataatataaatttcatgtatctgggagtggtcatatgaaaaggaattatatcttaggattagatatcggaattacatcagtgggttatggaattattgattatgaaactagagatgtcatagatgcgggcgtacgtttatttaaagaggctaatgttgaaaataatgaaggacgacgatcaaaaagaggtgccagaaggcttaagaggcgtcgtagacatagaatacaaagagtaaagaaacttttatttgattacaatttgttgacagatcatagtgagctaagtggaatcaatccttacgaggcgcgcgtaaagggattaagtcaaaaattaagtgaagaggaattttctgcggcattgctacatttagcaaagcgtagaggtgtacataatgttaatgaagtggaagaagatacaggtaatgaattatccactaaagaacaaatttcaagaaatagtaaagcgttagaagagaagtatgttgcagaattacagttggaacgtttgaaaaaagacggtgaagtgagaggttcgattaaccgtttcaaaacatctgactatgtaaaagaagcaaagcagttattaaaagtacaaaaagcatatcatcaacttgatcaatcatttatagacacttatattgatttattggaaacaagaagaacatattatgagggaccaggtgaaggtagcccatttggatggaaagatattaaagaatggtatgaaatgttaatgggacattgtacgtatttcccagaagaattacgtagtgtgaaatatgcctataatgctgatttatataatgcgctgaatgatttgaacaacttggttattacacgagatgagaatgagaagctagagtattatgaaaaattccaaattatcgagaatgtctttaaacaaaagaaaaagccgacgcttaaacaaattgcgaaggaaatcttggtgaatgaagaagacatcaaaggctatcgtgtcacaagtacaggtaaaccagaatttacaaacttgaaagtttatcacgatatcaaagatattacagcaagaaaagaaattatcgagaatgcagagctactcgatcaaatagctaaaatattaactatttaccagtcatcagaagatatacaagaagaattaacaaacctaaattcagaattgacacaagaagagattgaacaaatttcaaacttgaaaggttatacaggaactcataacctttcactaaaggcaataaatttaatattagacgaattgtggcatacgaacgataatcaaatagctattttcaatcgtttgaaacttgtacctaaaaaggtagatttaagccaacaaaaagaaattcctactactttagttgatgattttatactgtctccagtagtgaaacgttcatttatacaatctattaaagttattaacgctattattaaaaaatacggtttgccaaatgatattattattgaacttgcgagagaaaagaattctaaagatgcacaaaaaatgattaatgaaatgcagaagagaaatcgtcaaacgaatgaacgtattgaggaaattataagaacgacaggtaaagaaaatgctaaatatttaattgaaaaaattaagctgcacgatatgcaagaagggaaatgtttatactcgttagaagcaatccctctagaagatttacttaataatccattcaattacgaagtagaccatatcattccacgttctgtttctttcgataactctttcaataataaagtgttggtgaaacaagaagaaaatagtaaaaaaggtaatagaacgccatttcaatatttaagttcttcagattctaaaataagttatgagacattcaaaaagcatattttaaatcttgctaaaggcaaaggtagaatctctaagacgaaaaaagaatatttgttagaagaacgagatatcaatcgcttcagtgtccaaaaagattttattaaccgtaacttagtagatacacgctatgcgacaagagggttaatgaacttattaagatcttattttagagtgaataacttagatgtcaaagtgaaatcgattaatggcggattcacaagtttcttaagaaggaaatggaagttcaaaaaagaaagaaataagggctacaaacaccatgctgaagatgcactgattattgcgaacgctgattttattttcaaagaatggaaaaaactagataaagctaaaaaagtgatggaaaatcaaatgtttgaagaaaagcaagctgaaagtatgcctgaaattgagactgagcaagagtataaagaaatttttataacgcctcatcaaattaaacatattaaggattttaaagattataaatattcacatagagttgataaaaagccgaatagagagttaataaatgatacattatattctacgagaaaagatgacaagggtaatacattaatcgttaataacttaaatggtttatacgataaagataatgataaattgaaaaaattaattaataaatcacctgaaaaattattgatgtatcatcatgatccacaaacatatcaaaaattaaaattgatcatggaacaatatggcgatgagaaaaatccgctttataaatattatgaagaaacaggcaattacttaacaaaatatagtaaaaaagataacggaccagtcatcaaaaaaattaaatattatggtaacaagctaaatgcgcatttagatattacggatgattatccaaatagcagaaataaagtagtaaaactttcattaaaaccatatcgctttgatgtttatttagataatggggtatataaatttgtgacagttaaaaatttagatgttatcaaaaaagaaaactactatgaagttaattcaaagtgttatgaagaagcaaaaaaactgaagaaaattagtaatcaagcagaatttatcgcaagtttttacaataatgacttgattaagattaacggagaattatatagagtcataggtgtaaataatgatctacttaacagaattgaagtaaatatgatagacatcacatatagagaatatttagagaacatgaatgataaaagaccacctagaataattaaaacaatagcaagcaaaacacaatctattaaaaagtattctacagatattctaggcaatctttatgaagtgaagagtaaaaagcatcctcaaatcataaagaaaggatgattggatattggcatggagaattgtatatctttcagaagtagataagcttgcattaaatttaaataacttaaaagtcgcaaaaggggatttggaggtaaaaatcccccttagcgatattttcgcaattgtgattgaagatttaacaactactataacctctaggcttatgatagagctatctaaatacaatattttagtgattttttgtaatcaaaagcatttaccagagtgcatgattcaaccgattaatggtcattttaatcaatatggccaaatgaaggaacaactacaatggtcggaagaaagaaaagctgaattatggaaacatattctgtttcaaaaaatacaaaatcaaattcagtgtatgaaacattttggagtggatgaagaaagaataattaaaatgaaaaaattacaatcaatggttacatctaaagatgaaatgaatatagagggccaagcggctaagtattattttaatacatttttcaaggacttcagacgcgatgatgattttttagtagaaaatatggtactggattttgggtatactattttaaattcagcaatcgcaaggaccattgtagctaaagggttaattccagcattgggaatacatcatattggcgcaagaaaccactttaatttagcatcagatatcattgaagtatttaggccattggtagatttatatcttttgaaacatcctccgaaagtggaatatatgactagagagtatagattagagctgattaacttgctgcatgctagagtacaaattgatggaaagcagcatacagttattagagcgattgaaattatggttcaatcaataattgagtattttagaacggggagatataaaacgctcaaattaccaaatattaagcaatattcattttataaatcatgagttataagtttatgagagtaatgattatgtttgatctcccaactgacacaaaagaagaacgacggttatatagtaagtttagaaagggactcatttcggaaggctttttgatgatgcagtattctatttacattaaatgttgtattaataaagatgcggcaaatagtagtgtaaattatgtgaaacgtattttaccaccaaacggacatgttagagctttaacaattaccgaaaagcaatataaaaaaatgaaaatattattaggagatgaagataaaaatatcgaaatattaggagataatcgtacaattttattttaggagaaaacctatgtatgaatcaattttagaaatcaatattgatatggtacccaaagttattttaaatactagtgtatatacatctatatataatgaagattcaacacatgaagaatatattttagatatgcttaagaattattttcaatctagaaattcaaataaggatattgttacgattacagatatttcagatcatgaaagagtatctcataatcggtttagaggatttctcttagatcattctactattgaaaatgaacaccaattatcatcatcgagtattttgactaagaagattgttagagaaatgcaaagtgatttggaaatagatggttatattaattctatcaatgtactgttggatgacttacgagataatttaaagggcacactgccactttctattaagtctttcgatttaaaacaattcataaagctactctcatttaaatatgattattcggaagattatgccagactaattactcggttagaacaagtcgtcccattagtagtggatgaaatgaattatcaagtaaaagaaaaagcatttgtaatctatttatatccagaagctggcctaagcattaaagaacaaataagatttagaaaaatactaaataacttacctgttccggtcattgttctaaccgaatcaccacgttttttatctgaaagtattaaaggactaaattattttattaataatgttcaaatgatcacagaatctttttttgaagatagctattggaatgcaccaattaatgtagaaaaagaacagattgaagagaggtttgaatatttatttgtaaaatattgttcagttttagaaataaaaccgattatttctaactatttacttgcggatatcattgtttttaatgatattgatctttatatccttgtttcatttttgaaacactgtaatttagagtataaattagatatcgataaaacaaaaatttcattagcattatcgtcatatctattttcttaattattttgaggatttataatgatgctagaggttttagtactctgtaattttaggtatgaggtagaccaggtttgtacccactgacaccaacaagcggttttagtactctgtaattttaggtatgaggtagaccgtaaagactttaacgaatttatggataaagttttagtactctgtaattttaggtatgaggtagacaggaacaacctgatttaaatatgtggttgggttttagtactctgtaattttaggtatgaggtagactgtagcttcttcaagttctttaaatagttcgttttagtactctgtaattttaggtatgaggtagacaaagtggcgatgttattaatatcaaaggttgttttagtactctgtaattttaggtatgaggtagactaatgtttgcggtagaaggtttacctgtacgttttagtactctgtaattttaggtatgaggtagacaagttggtgaaattttatataacgcaaacagttttagtactctgtaattttaggtatgaggtagactaacgcatgtgtaatggttctaccctgccagttttagtactctgtaattttaggtatgaggtagacccactgcaacaagtcgtcgtgagcgtgtgcgttttagtactctgtaattttaggtatgaggtagacaaatataacgtggtttattacgtcagacgggttttagtactctgtaattttaggtatgaggtagacaaataccaaattttgaattgaacccaaatcgttttagtactctgtaattttaggtatgaggtatatcttttttaggtcggctttttattttgaatagttttagtactctgtaattttagatatgaggtatatagcaaaatcactgatagggagaggcgtatcataagtgatgagtttgtttattataagatatacgaaaaatattaatttaaagatatcagagaaacatagagtatttatataactgtttagaagtataaaataatcattttttgtatcatacagttggttctataatgaatcactaagaatgattgtattcaataaattaataaaaagcatatacatggtattagcaaatagaaattaactaggttttattggtttatagcctttaaataaatatatttaatttaaattcgcgattaggtagtagtaattaatgtttgagattgaaaatagatttaaatatagcaattatatattaacctattaaagtgttaggctataatgattagaatattctaggagatataaataaaatgaggaaattatacaatttaaaagaatttttaaatatttattcaactgaagatataggtttaattaatacatatatcgaatctgataatagaccacttaaagaaaatgaagtagaggatttaaaatcattaataaatctcttgaagctaaattataaaagttgtgaaggtttttttcttagttatgaagttcctcatatcggtcacgaaatagacttattgaaagttacggataatgctattttaaatatcgaattaaaaagtagatctgagcttgcaaagataaataaacaacaaaagtataattatttttatcttaatacacttaacaaaaatgtagacattataacctataatagacatgaagaaaagttttataaatattgtcaagaaagtgagaaatcacttgaaataaatatagataaagtaagggataaaatttttgaatatggaaataaagagtttatttcagatattgattatttatttaaaccttctaatttccttatttcaccttttaatgatactgacaaatttcttgaagacaaatattatttaacggcccagcaagaaaaaataaaaaaagacattataaatcataatgggactattgctattattgaaggaagaccaggcacaggtaaatcacttttattatatgatattgctaaaaaactaaaaaaagagtttaatatattaataatacattgtgcattgttaaatgaaggacacgaattaatgattaataaaaattggaatataaaaagtgctcataaaaattgggtatacgatgaagagaattatgaaggtaaaaattatatttttattgatgaatcacataggttttaccctaaacaatttgagtatgtaatagaaactgcacttaaaaaagatattaagataataacaactatagacccattacagtatctaagagataatgaaaatgattttgaaaacttacagagattaaaatctcattctaacatctattataaaaaaattgataataaaattagatctaatccagaaatatcatcatttgttaaaagtattattaatttaagaaatatacctgaatataaatttaagaatatttcaatagaatatttgtcaaaagaagatgattggaaatcatatttgctaaatttacgtgatagaggatggacatatttaccttatacgaaaagtagagataatattagttatcataaatattgttcggctaatactcatttaaatactcatagaattattgggcaagaatttaataaagttattgttattttagatgaaggatttaaatatgttgatggatatttaggatattacggagattattattataatcctagacaaatgttgttccaaaatttaactagagctagagaaaaaataaaaattataatcattaataatacagatttatataaaaagattaatcaagtgttaactaagtcttctaataaaaatgagttatcacttaaattttttattcctgaacttaataatgataaattaaaatcattttatagtgatattttaggttttaagttaattagtaatcaaaaacaaccgcctggaaaaagaaagataagttttcaaataggtgaaacaaatttagggttttatgaaaaaggagatatttctaaaaacaataaatgcgaaataaatatagttgtaagtaatttgaaagatttaaagaaaagaatatcaaatgaaaatatggtattgattagtgaagaagaaggtaaaaaaagtaaatttgttactttaaatgatccattaaacaactatttaaagttaatagagtatatataactagtattttgaattatttaaagatttattgaagttttgatattaatttgtcgaaaaacgaaccaaattattaaatgctacacaaaagaatatcaagtataagttattaatcataaatcagattgggtactcacctattggaagtgaagatgccaaactattattccaattaatagatttaaggtatgagaagaaaagtacaatagttaccacaaatatcaaattcaacttatgtaacgaaatatttgatgattccaaaatcgcaaatgcgattttggataggatattgcatcattcaagcgtagttaaaatcacaggtaaatcatatagattaaaagatcattcacctaagaaggaaattacttagcaaacaattttgtacattcttatacaatcatttatgtacatttttatattgacatttacaagtaagcaagtgaacttatctgctccagctgtaagagaaagggtaaataaacttgaagagcaaggtattatacaaggttatacaattaacatagattataaacaattaggttacgatgtagaaaaattaattgagttaactataaagaataatagatacagccatatgggcagacaaaatgtcagtttatcttttcatcagttgtctaaactacatggaaaaagtttaataagcataggaaagatttttaacagagagaagtgacttattttggaatataaatcttacaacaaaatgagtaataatattttatctatcttgttaagtgaaaaaaatttcgataataaaatggtagtctcaacaggtagttatattttgtctgagttgccatgtattgttgcctataaaaataatgatattgtggggctactaacgtataaagtttatgatgagtacattgaaatcatttctttagatagttttgtagagaacaagggtattggtagtcatttacttaattatgctgaaataattgcctcagatatgagtaaaagaagtatccgtgttattactacaaatgaaaatattaaggcactctatttctatcaaaaaaataaatatagaatcacagacgttatttttgatgctgtaacagaagctaggaaaataaagccgtcgattcctacaattgataaaaatggcattgaaattagagatgaaattgttttgaggaaatgtttgtaatgtataaatacactcagctttaaatcaccctagttcatacctaaaagactttaacacaaacaaaaaaggaggaacattaaattcctcctcaacctttattactcatactacaattctattttaacgtcttcgtccatttgggcttcaaattcatctagaagtgctcttgcttctgcaattgattgtgtgttcatcaattgatggcgaagttcgctagcgcctcttatgccacgcacatagattttaaagaatctacgcaagctcttgaattgtcgtatttcatctttctcatatttgttaaacaatgatagatgcaatctcaacagatctaatagttctttgcttgtgtgttcacgtggttctttttcaaaagcgaatggattgtggaaaatgcctctaccaatcatgacgccatcaatgccatatttttctgccagttcaagtcctgtttttctatcgggaatatcaccgttaattgttaacaatgtatttggtgcaatttcgtcacgtaaatttttaatagcttcgattaattcccaatgtgcatctactttactcatttctttacgtgtacgaagatgaatagataaattggcaatgtcttgttcgaagacgtgcttcaaccaatctttccattcatcgatttcatagtagccaaggcgtgttttaacacttaccggaagcccacctgctttagtcgcttgaataatttcggcagcaacgtcaggtcttaagattaagccggaacccttaccctttttagcaacatttgctacaggacatcccatatttaagtctatgcctttaaagcccattttagctaattgaatactcgtttcacggaactgttctggcttatctccccatatatgagcgaccatcggctgttcatcttcactaaaagttaagcgtccgcgcacactatgtatgccttcagggtggcaaaagctttcagtatttgtaaattcagtgaaaaacacatccggtctagctgcttcacttacaacgtgtcgaaagacgatatctgtaacgtcttccattggcgccaaaataaaaaatggacgtggtaattcactccaaaaattttctttcataatatatttataccctct

SEQ ID NO: 50 - DNA, 23 bp, unidentified
  source 1..23: mol_type = other DNA; note = Bacterial
cctggcctgccccaagtgcaagg

SEQ ID NO: 51 - DNA, 32 bp, unidentified
  source 1..32: mol_type = other DNA; note = Bacterial
gtcgccccccacgcgggggcgtggattgaaac

SEQ ID NO: 52 - DNA, 28 bp, unidentified
  source 1..28: mol_type = other DNA; note = Bacterial
tggagcgggaaacgggatttgaacccgc

SEQ ID NO: 53 - DNA, 29 bp, unidentified
  source 1..29: mol_type = other DNA; note = Bacterial
gtgttccccacgggcgtggggatgaaccg

SEQ ID NO: 54 - DNA, 25 bp, unidentified
  source 1..25: mol_type = other DNA; note = Bacterial
aacctttctgcaaaaaggtttcccc

SEQ ID NO: 55 - DNA, 23 bp, unidentified
  source 1..23: mol_type = other DNA; note = Bacterial
ccgctggatccggctgcagcgcc

SEQ ID NO: 56 - DNA, 28 bp, unidentified
  source 1..28: mol_type = other DNA; note = Bacterial
gttcactgccgcataggcagctcagaaa

SEQ ID NO: 57 - DNA, 32 bp, unidentified
  source 1..32: mol_type = other DNA; note = Bacterial
cacccgactattgaagtcgggcctcattgaag

SEQ ID NO: 58 - DNA, 36 bp, unidentified
  source 1..36: mol_type = other DNA; note = Bacterial
gtcaaaacccataccgatatggatacctcttttgag

SEQ ID NO: 59 - DNA, 36 bp, unidentified; identical to SEQ ID NO: 58
  source 1..36: mol_type = other DNA; note = Bacterial

SEQ ID NO: 60 - DNA, 36 bp, unidentified; identical to SEQ ID NO: 58
  source 1..36: mol_type = other DNA; note = Bacterial

SEQ ID NO: 61 - DNA, 36 bp, unidentified; identical to SEQ ID NO: 58
  source 1..36: mol_type = other DNA; note = Bacterial

SEQ ID NO: 62 - DNA, 36 bp, unidentified
  source 1..36: mol_type = other DNA; note = Bacterial
ctcaaaagaggtatccatatcggtatgggttttgac

SEQ ID NO: 63 - DNA, 28 bp, unidentified
  source 1..28: mol_type = other DNA; note = Bacterial
gttcactgccggataggcagcttagaaa

SEQ ID NO: 64 - DNA, 32 bp, unidentified
  source 1..32: mol_type = other DNA; note = Bacterial
gtcgccccctgcgcgggggcgtggattgaaac

SEQ ID NO: 65 - DNA, 29 bp, unidentified
  source 1..29: mol_type = other DNA; note = Bacterial
ttttctgagctgcctatgcggcagtgaac

SEQ ID NO: 66 - DNA, 46 bp, unidentified
  source 1..46: mol_type = other DNA; note = Bacterial
catcgacgacgaacccgggcaccgcctgatggtccacgccgtcatg

SEQ ID NO: 67 - DNA, 32 bp, unidentified
  source 1..32: mol_type = other DNA; note = Bacterial
gtcgcccctcacgcgggggcgtggatagaaac

SEQ ID NO: 68 - DNA, 32 bp, unidentified
  source 1..32: mol_type = other DNA; note = Bacterial
gtttcaatccacgcccccgcacggggggcgac

SEQ ID NO: 69 - DNA, 28 bp, unidentified
  source 1..28: mol_type = other DNA; note = Bacterial
tttctgagctgcctatgcggcagtgaac

SEQ ID NO: 70 - DNA, 36 bp, unidentified
  source 1..36: mol_type = other DNA; note = Bacterial
gaccgaagacctgtcggaaacgacggggattgagac

SEQ ID NO: 71 - DNA, 29 bp, unidentified
  source 1..29: mol_type = other DNA; note = Bacterial
cggttcatccccgcgagtgcggggaacat

SEQ ID NO: 72 - DNA, 28 bp, unidentified
  source 1..28: mol_type = other DNA; note = Bacterial
tttctgagctgcctgtgcggcagtgaac

SEQ ID NO: 73 - DNA, 29 bp, unidentified
  source 1..29: mol_type = other DNA; note = Bacterial
gttttatctgaacgtagtgggatataaag

SEQ ID NO: 74 - DNA, 29 bp, unidentified
  source 1..29: mol_type = other DNA; note = Bacterial
cggttcatccccgcgggtgcggggaacac

SEQ ID NO: 75 - DNA, 28 bp, unidentified
  source 1..28: mol_type = other DNA; note = Bacterial
gttagcagccgcataggctgcttaaata

SEQ ID NO: 76 - DNA, 33 bp, unidentified
  source 1..33: mol_type = other DNA; note = Bacterial
aatttaaatagggaagataagcaaagggttgac

SEQ ID NO: 77 - DNA, 31 bp, unidentified
  source 1..31: mol_type = other DNA; note = Bacterial
tttaaatagggaagataagcaaagggttgac

SEQ ID NO: 78 - protein, 11 aa, unidentified
  source 1..11: note = Bacterial
NLNREDKQRVD

SEQ ID NO: 79 - DNA, 32 bp, unidentified
  source 1..32: mol_type = other DNA; note = Bacteriophage
cattgcaactatgcaaaatgatgaagctaaaa

SEQ ID NO: 80 - DNA, 32 bp, unidentified
  source 1..32: mol_type = other DNA; note = Bacteriophage
tgttagagtcggtagtatctggatgatcgata

SEQ ID NO: 81 - DNA, 32 bp, unidentified
  source 1..32: mol_type = other DNA; note = Bacteriophage
ttatgtattgaccccgacacgccccccgactg

SEQ ID NO: 82 - DNA, 32 bp, unidentified
  source 1..32: mol_type = other DNA; note = Bacteriophage
ttacagacgacctaactcttcagtaccatgat

SEQ ID NO: 83 - DNA, 32 bp, unidentified
  source 1..32: mol_type = other DNA; note = Bacteriophage
tacataagctgcaacacggtgttcgtttaagt

SEQ ID NO: 84 - DNA, 32 bp, unidentified
  source 1..32: mol_type = other DNA; note = Bacteriophage
aaaatacgcctttttcccttcatcgtttaaag

SEQ ID NO: 85 - DNA, 32 bp, unidentified
  source 1..32: mol_type = other DNA; note = Bacteriophage
accaacaaatcccataaactgataaccacgtt

SEQ ID NO: 86 - DNA, 32 bp, unidentified
  source 1..32: mol_type = other DNA; note = Bacteriophage
gtcaaccctttgcttatcttccctatttaaat

SEQ ID NO: 87 - DNA, 32 bp, unidentified
  source 1..32: mol_type = other DNA; note = Bacteriophage
tgttaaccaccgcttgaaataatcatgatgca

SEQ ID NO: 88 - DNA, 32 bp, unidentified
  source 1..32: mol_type = other DNA; note = Bacteriophage
tgtgtctatactcaaccaatttaagcgccgca

SEQ ID NO: 89 - DNA, 32 bp, unidentified
  source 1..32: mol_type = other DNA; note = Bacteriophage
ctactctccccaatattagccattcctaattc

SEQ ID NO: 90 - DNA, 32 bp, unidentified
  source 1..32: mol_type = other DNA; note = Bacteriophage
gtcaccttaccgtaagacaggcagtaaaatta

SEQ ID NO: 91 - DNA, 32 bp, unidentified
  source 1..32: mol_type = other DNA; note = Bacteriophage
aaactagtggacgtaatgcagtattcacggtt

SEQ ID NO: 92 - DNA, 32 bp, unidentified
  source 1..32: mol_type = other DNA; note = Bacteriophage
atccacactacaaatagaacactcaaccgtga

SEQ ID NO: 93 - DNA, 32 bp, unidentified; identical to SEQ ID NO: 88
  source 1..32: mol_type = other DNA; note = Bacteriophage

SEQ ID NO: 94 - DNA, 32 bp, unidentified; identical to SEQ ID NO: 89
  source 1..32: mol_type = other DNA; note = Bacteriophage

SEQ ID NO: 95 - DNA, 32 bp, unidentified; identical to SEQ ID NO: 91
  source 1..32: mol_type = other DNA; note = Bacteriophage

SEQ ID NO: 96 - DNA, 32 bp, unidentified
  source 1..32: mol_type = other DNA; note = Bacteriophage
ataatcgttttgagtctcaccagcttttaggc

SEQ ID NO: 97 - DNA, 32 bp, unidentified; identical to SEQ ID NO: 92
  source 1..32: mol_type = other DNA; note = Bacteriophage

SEQ ID NO: 98 - DNA, 32 bp, unidentified
  source 1..32: mol_type = other DNA; note = Bacteriophage
tattgattggtctctaaccttgggatgattaa

SEQ ID NO: 99 - DNA, 32 bp, unidentified
  source 1..32: mol_type = other DNA; note = Bacteriophage
ttcacgggtagcaacagggtaataaaccaata

SEQ ID NO: 100 - DNA, 32 bp, unidentified; identical to SEQ ID NO: 79
  source 1..32: mol_type = other DNA; note = Bacteriophage

SEQ ID NO: 101 - DNA, 32 bp, unidentified; identical to SEQ ID NO: 80
  source 1..32: mol_type = other DNA; note = Bacteriophage

SEQ ID NO: 102 - DNA, 32 bp, unidentified
  source 1..32: mol_type = other DNA; note = Bacteriophage
tagaagagtaataggagctactgcaaacttgt

SEQ ID NO: 103 - DNA, 32 bp, unidentified
  source 1..32: mol_type = other DNA; note = Bacteriophage
taactatgtgtggtttatattttgtgtgcaag

SEQ ID NO: 104 - DNA, 32 bp, unidentified
  source 1..32: mol_type = other DNA; note = Bacteriophage
ttttgaaactattgacagaaggttgggaacct

SEQ ID NO: 105 - DNA, 32 bp, unidentified
  source 1..32: mol_type = other DNA; note = Bacteriophage
ttgaggttgaacctcttccggttcctcttctg

SEQ ID NO: 106 - DNA, 32 bp, unidentified
  source 1..32: mol_type = other DNA; note = Bacteriophage
gtgtattgcttgcagtgggttacacacaagaa

SEQ ID NO: 107 - DNA, 47 bp, unidentified
  source 1..47: mol_type = other DNA; note = Bacterial
gttgtgatttgctttcaaattagtatctttgaaccattggaaacagc

SEQ ID NO: 108 - DNA, 29 bp, unidentified
  source 1..29: mol_type = other DNA; note = Bacterial
atttcaattccataaggtacaattaatac

SEQ ID NO: 109 - DNA, 32 bp, unidentified
  source 1..32: mol_type = other DNA; note = Bacterial
gtttcaatccacacacccgtatagggtgtgac

SEQ ID NO: 110 - DNA, 47 bp, unidentified
  source 1..47: mol_type = other DNA; note = Bacterial
actgtttctgatatgtcaaagataaaattttgaaagcaaatcacaac

SEQ ID NO: 111 - DNA, 23 bp, unidentified
  source 1..23: mol_type = other DNA; note = Bacterial
gaaaaaatacagtttcgctctca

SEQ ID NO: 112 - DNA, 32 bp, unidentified
  source 1..32: mol_type = other DNA; note = Bacterial
gtcgcgtctcacgtaggcgcgtggattgaaac

SEQ ID NO: 113 - DNA, 47 bp, unidentified
  source 1..47: mol_type = other DNA; note = Bacterial
attgtgcttgctactgcaaagatacacattttgaagcaattcacaac

SEQ ID NO: 114 - DNA, 37 bp, unidentified
  source 1..37: mol_type = other DNA; note = Bacterial
ctcaatgagtatcttccattaaaacaaggattaagac

SEQ ID NO: 115 - DNA, 36 bp, unidentified
  source 1..36: mol_type = other DNA; note = Bacterial
gttgtttttaccttgcaaacagcaggcagatacaac

SEQ ID NO: 116 - DNA, 47 bp, unidentified
  source 1..47: mol_type = other DNA; note = Bacterial
gttgtatttgccaatgcaaagatactaattttaaagctaatcacaac

SEQ ID NO: 117 - DNA, 36 bp, unidentified
  source 1..36: mol_type = other DNA; note = Bacterial
gttgtatatcattcctttcctacatcaaaccacaac

SEQ ID NO: 118 - DNA, 487 bp, synthetic construct
  source 1..487: mol_type = other DNA
gcggataacaattactagagaaagaggagaaatactattcttctcctctttaaataacgaaaacaccctgccataaaatgacagggtgttgatttcggcatgaagccttatctttgtagcttctgcaagatttaagtaactgtgtaaggcgtcccttacacttgcatgtatagttattataccagggggacagtgcaatgtcaagaataaactgtagaatgactagtgacttaaatcttgagagtacaaaaacccgttggaatcgtgattaatagtaactgttgttgtacagttacttaaatcttgagagtacaaaaacggccgagaaaaggagctgattcataggacagttgtacagttacttaaatcttgagagtacaaaaactcaaacttgcccgtagtttatcttatagccgttgtacagttacttaaatcttgagagtacaaaaacatttacctcctttgatttaagtgaacaagtttatcc

SEQ ID NO: 119 - DNA, 221 bp, Streptococcus thermophilus
  source 1..221: mol_type = other DNA
ttaaatcttgagagtacaaaaacccgttggaatcgtgattaatagtaactgttgttgtacagttacttaaatcttgagagtacaaaaacggccgagaaaaggagctgattcataggacagttgtacagttacttaaatcttgagagtacaaaaactcaaacttgcccgtagtttatcttatagccgttgtacagttacttaaatcttgagagtacaaaaac

SEQ ID NO: 120 - DNA, 112 bp, Streptococcus thermophilus
  source 1..112: mol_type = other DNA
ttaaataacgaaaacaccctgccataaaatgacagggtgttgatttcggcatgaagccttatctttgtagcttctgcaagatttaagtaactgtgtaaggcgtcccttacac

SEQ ID NO: 121 - DNA, 30 bp, Streptococcus thermophilus
  source 1..30: mol_type = other DNA
tgtcctatgaatcagctccttttctcggcc

SEQ ID NO: 122 - DNA, 30 bp, Streptococcus thermophilus
  source 1..30: mol_type = other DNA
ggctataagataaactacgggcaagtttga